European Patent Application EP 4 549 455 A1, published May 7, 2025. Title: MODIFIED FUSION PROTEIN AND THE USE THEREOF. Applicant: 주식회사 파노로스바이오사이언스. The sequence listing filed with the application follows.

SEQUENCE LISTING (101 sequences)

SEQ ID NO: 1 - protein, 1338 aa, Homo sapiens
MVSYWDTGVLLCALLSCLLLTGSSSGSKLKDPELSLKGTQHIMQAGQTLHLQCRGEAAHKWSLPEMVSKESERLSITKSACGRNGKQFCSTLTLNTAQANHTGFYSCKYLAVPTSKKKETESAIYIFISDTGRPFVEMYSEIPEIIHMTEGRELVIPCRVTSPNITVTLKKFPLDTLIPDGKRIIWDSRKGFIISNATYKEIGLLTCEATVNGHLYKTNYLTHRQTNTIIDVQISTPRPVKLLRGHTLVLNCTATTPLNTRVQMTWSYPDEKNKRASVRRRIDQSNSHANIFYSVLTIDKMQNKDKGLYTCRVRSGPSFKSVNTSVHIYDKAFITVKHRKQQVLETVAGKRSYRLSMKVKAFPSPEVVWLKDGLPATEKSARYLTRGYSLIIKDVTEEDAGNYTILLSIKQSNVFKNLTATLIVNVKPQIYEKAVSSFPDPALYPLGSRQILTCTAYGIPQPTIKWFWHPCNHNHSEARCDFCSNNEESFILDADSNMGNRIESITQRMAIIEGKNKMASTLVVADSRISGIYICIASNKVGTVGRNISFYITDVPNGFHVNLEKMPTEGEDLKLSCTVNKFLYRDVTWILLRTVNNRTMHYSISKQKMAITKEHSITLNLTIMNVSLQDSGTYACRARNVYTGEEILQKKEITIRDQEAPYLLRNLSDHTVAISSSTTLDCHANGVPEPQITWFKNNHKIQQEPGIILGPGSSTLFIERVTEEDEGVYHCKATNQKGSVESSAYLTVQGTSDKSNLELITLTCTCVAATLFWLLLTLFIRKMKRSSSEIKTDYLSIIMDPDEVPLDEQCERLPYDASKWEFARERLKLGKSLGRGAFGKVVQASAFGIKKSPTCRTVAVKMLKEGATASEYKALMTELKILTHIGHHLNVVNLLGACTKQGGPLMVIVEYCKYGNLSNYLKSKRDLFFLNKDAALHMEPKKEKMEPGLEQGKKPRLDSVTSSESFASSGFQEDKSLSDVEEEEDSDGFYKEPITMEDLISYSFQVARGMEFLSSRKCIHRDLAARNILLSENNVVKICDFGLARDIYKNPDYVRKGDTRLPLKWMAPESIFDKIYSTKSDVWSYGVLLWEIFSLGGSPYPGVQMDEDFCSRLREGMRMRAPEYSTPEIYQIMLDCWHRDPKERPRFAELVEKLGDLLQANVQQDGKDYIPINAILTGNSGFTYSTPAFSEDFFKESISAPKFNSGSSDDVRYVNAFKFMSLERIKTFEELLPNATSMFDDYQGDSSTLLASPMLKRFTWTDSKPKASLKIDLRVTSKSKESGLSDVSRPSFCHSSCGHVSEGKRRFTYDHAELERKIACCSPPPDYNSVVLYSTPPI

SEQ ID NO: 2 - protein, 432 aa, synthetic construct
EFGRPFVEMYSEIPEIIHMTEGRELVIPCRVTSPNITVTLKKFPLDTLIPDGKRIIWDSRKGFIISNATYKEIGLLTCEATVNGHLYKTNYLTHRQTNTIIDVQISTPSPVTLLRGHTLVLNCTATTPLNTRVQMTWSYPDEKNKRASVRRRIDQSNSHANIFYSVLTIDKMQNKDKGLYTCRVRSGPSFKSVNTSVHIYDKALEDKTHTCPPCPAPELLGGPSVFLFPPKPKDTLMISRTPEVTCVVVDVSHEDPEVKFNWYVDGVEVHNAKTKPREEQYNSTYRVVSVLTVLHQDWLNGKEYKCKVSNKALPAPIEKTISKAKGQPREPQVYTLPPSREEMTKNQVSLTCLVKGFYPSDIAVEWESNGQPENNYKTTPPVLDSDGSFFLYSKLTVDKSRWQQGNVFSCSVMHEALHNHYTQKSLSLSPGK

SEQ ID NO: 3 - protein, 432 aa, synthetic construct
EFGRPFVEMYSEIPEIIHMTEGRELVIPCRVTSPNITVTLKKFPLDTLIPDGKRIIWDSRKGFIISNATYKEIGLLTCEATVNGHLYKTNYLTHRQTNTIIDVQISTPSPVTLLRGHTLVLNCTATTPLNTRVQMTWSYPDEKNKNASVRRRIDQSNSHANIFYSVLTIDKMQNKDKGLYTCRVRSGPSFKSVNTSVHIYDKALEDKTHTCPPCPAPELLGGPSVFLFPPKPKDTLMISRTPEVTCVVVDVSHEDPEVKFNWYVDGVEVHNAKTKPREEQYNSTYRVVSVLTVLHQDWLNGKEYKCKVSNKALPAPIEKTISKAKGQPREPQVYTLPPSREEMTKNQVSLTCLVKGFYPSDIAVEWESNGQPENNYKTTPPVLDSDGSFFLYSKLTVDKSRWQQGNVFSCSVMHEALHNHYTQKSLSLSPGK

SEQ ID NO: 4 - protein, 428 aa, synthetic construct
EFGRPFVEMYSEIPEIIHMTEGRELVIPCRVTSPNITVTLKKFPLDTLIPDGKRIIWDSRKGFIISNATYKEIGLLTCEATVNGHLYKTNYLTHRQTNTIIDVQISTPSPVTLLRGHTLVLNCTATTPLNTRVQMTWSYPDEKNKNASVRRRIDQSNSHANIFYSVLTIDKMQNKDKGLYTCRVRSGPSFKSVNTSVHIYDKDKTHTCPPCPAPELLGGPSVFLFPPKPKDTLMISRTPEVTCVVVDVSHEDPEVKFNWYVDGVEVHNAKTKPREEQYNSTYRVVSVLTVLHQDWLNGKEYKCKVSNKALPAPIEKTISKAKGQPREPQVYTLPPSREEMTKNQVSLTCLVKGFYPSDIAVEWESNGQPENNYKTTPPVLDSDGSFFLYSKLTVDKSRWQQGNVFSCSVMHEALHNHYTQKSLSLSPG

SEQ ID NO: 5 - protein, 426 aa, synthetic construct
EFGRPFVEMYSEIPEIIHMTEGRELVIPCRVTSPNITVTLKKFPLDTLIPDGKRIIWDSRKGFIISNATYKEIGLLTCEATVNGHLYKTNYLTHRQTNTIIDVQISTPSPVTLLRGHTLVLNCTATTPLNTRVQMTWSYPDEKNKNASVRRRIDQSNSHANIFYSVLTIDKMQNKDKGLYTCRVRSGPSFKSVNTSVHIYDKETKTPECPAPELLGGPSVFLFPPKPKDTLMISRTPEVTCVVVDVSHEDPEVKFNWYVDGVEVHNAKTKPREEQYNSTYRVVSVLTVLHQDWLNGKEYKCKVSNKALPAPIEKTISKAKGQPREPQVYTLPPSREEMTKNQVSLTCLVKGFYPSDIAVEWESNGQPENNYKTTPPVLDSDGSFFLYSKLTVDKSRWQQGNVFSCSVMHEALHNHYTQKSLSLSPG

SEQ ID NO: 6 - protein, 429 aa, synthetic construct
SDTGRPFVEMYSEIPEIIHMTEGRELVIPCRVTSPNITVTLKKFPLDTLIPDGKRIIWDSRKGFIISNATYKEIGLLTCEATVNGHLYKTNYLTHRQTNTIIDVQISTPSPVTLLRGHTLVLNCTATTPLNTRVQMTWSYPDEKNKNASVRRRIDQSNSHANIFYSVLTIDKMQNKDKGLYTCRVRSGPSFKSVNTSVHIYDKDKTHTCPPCPAPELLGGPSVFLFPPKPKDTLMISRTPEVTCVVVDVSHEDPEVKFNWYVDGVEVHNAKTKPREEQYNSTYRVVSVLTVLHQDWLNGKEYKCKVSNKALPAPIEKTISKAKGQPREPQVYTLPPSREEMTKNQVSLTCLVKGFYPSDIAVEWESNGQPENNYKTTPPVLDSDGSFFLYSKLTVDKSRWQQGNVFSCSVMHEALHNHYTQKSLSLSPG

SEQ ID NO: 7 - protein, 427 aa, synthetic construct
SDTGRPFVEMYSEIPEIIHMTEGRELVIPCRVTSPNITVTLKKFPLDTLIPDGKRIIWDSRKGFIISNATYKEIGLLTCEATVNGHLYKTNYLTHRQTNTIIDVQISTPSPVTLLRGHTLVLNCTATTPLNTRVQMTWSYPDEKNKNASVRRRIDQSNSHANIFYSVLTIDKMQNKDKGLYTCRVRSGPSFKSVNTSVHIYDKETKTPECPAPELLGGPSVFLFPPKPKDTLMISRTPEVTCVVVDVSHEDPEVKFNWYVDGVEVHNAKTKPREEQYNSTYRVVSVLTVLHQDWLNGKEYKCKVSNKALPAPIEKTISKAKGQPREPQVYTLPPSREEMTKNQVSLTCLVKGFYPSDIAVEWESNGQPENNYKTTPPVLDSDGSFFLYSKLTVDKSRWQQGNVFSCSVMHEALHNHYTQKSLSLSPG

SEQ ID NO: 8 - protein, 426 aa, synthetic construct
GRPFVEMYSEIPEIIHMTEGRELVIPCRVTSPNITVTLKKFPLDTLIPDGKRIIWDSRKGFIISNATYKEIGLLTCEATVNGHLYKTNYLTHRQTNTIIDVQISTPSPVTLLRGHTLVLNCTATTPLNTRVQMTWSYPDEKNKNASVRRRIDQSNSHANIFYSVLTIDKMQNKDKGLYTCRVRSGPSFKSVNTSVHIYDKDKTHTCPPCPAPELLGGPSVFLFPPKPKDTLMISRTPEVTCVVVDVSHEDPEVKFNWYVDGVEVHNAKTKPREEQYNSTYRVVSVLTVLHQDWLNGKEYKCKVSNKALPAPIEKTISKAKGQPREPQVYTLPPSREEMTKNQVSLTCLVKGFYPSDIAVEWESNGQPENNYKTTPPVLDSDGSFFLYSKLTVDKSRWQQGNVFSCSVMHEALHNHYTQKSLSLSPG

SEQ ID NO: 9 - protein, 424 aa, synthetic construct
GRPFVEMYSEIPEIIHMTEGRELVIPCRVTSPNITVTLKKFPLDTLIPDGKRIIWDSRKGFIISNATYKEIGLLTCEATVNGHLYKTNYLTHRQTNTIIDVQISTPSPVTLLRGHTLVLNCTATTPLNTRVQMTWSYPDEKNKNASVRRRIDQSNSHANIFYSVLTIDKMQNKDKGLYTCRVRSGPSFKSVNTSVHIYDKETKTPECPAPELLGGPSVFLFPPKPKDTLMISRTPEVTCVVVDVSHEDPEVKFNWYVDGVEVHNAKTKPREEQYNSTYRVVSVLTVLHQDWLNGKEYKCKVSNKALPAPIEKTISKAKGQPREPQVYTLPPSREEMTKNQVSLTCLVKGFYPSDIAVEWESNGQPENNYKTTPPVLDSDGSFFLYSKLTVDKSRWQQGNVFSCSVMHEALHNHYTQKSLSLSPG

SEQ ID NO: 10 - protein, 429 aa, synthetic construct
EFGRPFVEMYSEIPEIIHMTEGRELVIPCRVTSPNITVTLKKFPLDTLIPDGKRIIWDSRKGFIISNATYKEIGLLTCEATVNGHLYKTNYLTHRQTNTIIDVQISTPSPVTLLRGHTLVLNCTATTPLNTRVQMTWSYPDEKNKNASVRRRIDQSNSHANIFYSVLTIDGMQNKDKGLYTCRVRSGPSFKSVNTSVHIYDEDKTHTCPPCPAPELLGGPSVFLFPPKPKDTLMISRTPEVTCVVVDVSHEDPEVKFNWYVDGVEVHNAKTKPREEQYNSTYRVVSVLTVLHQDWLNGKEYKCKVSNKALPAPIEKTISKAKGQPREPQVYTLPPSREEMTKNQVSLTCLVKGFYPSDIAVEWESNGQPENNYKTTPPVLDSDGSFFLYSKLTVDKSRWQQGNVFSCSVMHEALHNHYTQKSLSLSPGK

SEQ ID NO: 11 - protein, 429 aa, synthetic construct
EFGRPFVEMYSEIPEIIHMTEGRELVIPCRVTSPNITVTLKKFPLDTLIPDGKRIIWDSRKGFIISNATYKEIGLLTCEATVNGHLYKTNYLTHRQTNTIIDVQISTPSPVTLSVGHTLVLNCTATTPLNTRVQMTWSYPDEKNKNASVRRRIDQSNSHANIFYSVLTIDKMQNKDKGLYTCRVRSGPSFKSVNTSVHIYDEDKTHTCPPCPAPELLGGPSVFLFPPKPKDTLMISRTPEVTCVVVDVSHEDPEVKFNWYVDGVEVHNAKTKPREEQYNSTYRVVSVLTVLHQDWLNGKEYKCKVSNKALPAPIEKTISKAKGQPREPQVYTLPPSREEMTKNQVSLTCLVKGFYPSDIAVEWESNGQPENNYKTTPPVLDSDGSFFLYSKLTVDKSRWQQGNVFSCSVMHEALHNHYTQKSLSLSPGK

SEQ ID NO: 12 - protein, 429 aa, synthetic construct
EFGRPFVEMYSEIPEIIHMTEGRELVIPCRVTSPNITVTLKKFPLDTLIPDGKRIIWDSRKGFIISNATYKEIGLLTCEATVNGHLYKTNYLTHRQTNTIIDVQISTPSPVTLSVGHTLVLNCTATTPLNTRVQMTWSYPDEKNKNASVRRRIDQSNSHANIFYSVLTIDGMQNKDKGLYTCRVRSGPSFKSVNTSVHIYDEDKTHTCPPCPAPELLGGPSVFLFPPKPKDTLMISRTPEVTCVVVDVSHEDPEVKFNWYVDGVEVHNAKTKPREEQYNSTYRVVSVLTVLHQDWLNGKEYKCKVSNKALPAPIEKTISKAKGQPREPQVYTLPPSREEMTKNQVSLTCLVKGFYPSDIAVEWESNGQPENNYKTTPPVLDSDGSFFLYSKLTVDKSRWQQGNVFSCSVMHEALHNHYTQKSLSLSPGK

SEQ ID NO: 13 - protein, 429 aa, synthetic construct
EFGRPFVEMYSEIPEIIHMTEGRELVIPCRVTSPNITVTLKKFPLDTLIPDGKRIIWDSRKGFIISNATYKEIGLLTCEATVNGHLYKTNYLTHRQTNTIIDVQISTPSPVELSVGETLVLNCTATTPLNTRVQMTWSYPDEKNKNASVRRRIDQSNSHANIFYSVLTIDKMQNKDKGLYTCRVRSGPSFKSVNTSVHIYDEDKTHTCPPCPAPELLGGPSVFLFPPKPKDTLMISRTPEVTCVVVDVSHEDPEVKFNWYVDGVEVHNAKTKPREEQYNSTYRVVSVLTVLHQDWLNGKEYKCKVSNKALPAPIEKTISKAKGQPREPQVYTLPPSREEMTKNQVSLTCLVKGFYPSDIAVEWESNGQPENNYKTTPPVLDSDGSFFLYSKLTVDKSRWQQGNVFSCSVMHEALHNHYTQKSLSLSPGK

SEQ ID NO: 14 - protein, 429 aa, synthetic construct
EFGRPFVEMYSEIPEIIHMTEGRELVIPCRVTSPNITVTLKKFPLDTLIPDGKRIIWDSRKGFIISNATYKEIGLLTCEATVNGHLYKTNYLTHRQTNTIIDVQISTPSPVELSVGETLVLNCTATTPLNTRVQMTWSYPDEKNKNASVRRRIDQSNSHANIFYSVLTIDGMQNKDKGLYTCRVRSGPSFKSVNTSVHIYDEDKTHTCPPCPAPELLGGPSVFLFPPKPKDTLMISRTPEVTCVVVDVSHEDPEVKFNWYVDGVEVHNAKTKPREEQYNSTYRVVSVLTVLHQDWLNGKEYKCKVSNKALPAPIEKTISKAKGQPREPQVYTLPPSREEMTKNQVSLTCLVKGFYPSDIAVEWESNGQPENNYKTTPPVLDSDGSFFLYSKLTVDKSRWQQGNVFSCSVMHEALHNHYTQKSLSLSPGK

SEQ ID NO: 15 - protein, 429 aa, synthetic construct
EFGRPFVEMYSEIPEIIHMTEGRELVIPCRVTSPNITVTLKKFPLDTLIPDGKRIIWDSRKGFIISNATYKEIGLLTCEATVNGHLYKTNYLTHRQTNTIIDVQISTPSPVTLLRGHTLVLNCTATTPLNTRVQMTWSYPDEKNKNASVRRRIDQSNSHANIFYSVLTIDGMTNSDKGLYTCRVRSGPSFKSVNTSVHIYDEDKTHTCPPCPAPELLGGPSVFLFPPKPKDTLMISRTPEVTCVVVDVSHEDPEVKFNWYVDGVEVHNAKTKPREEQYNSTYRVVSVLTVLHQDWLNGKEYKCKVSNKALPAPIEKTISKAKGQPREPQVYTLPPSREEMTKNQVSLTCLVKGFYPSDIAVEWESNGQPENNYKTTPPVLDSDGSFFLYSKLTVDKSRWQQGNVFSCSVMHEALHNHYTQKSLSLSPGK

SEQ ID NO: 16 - protein, 429 aa, synthetic construct
EFGRPFVEMYSEIPEIIHMTEGRELVIPCRVTSPNITVTLKKFPLDTLIPDGKRIIWDSRKGFIISNATYKEIGLLTCEATVNGHLYKTNYLTHRQTNTIIDVQISTPSPVTLLRGHTLVLNCTATTPLNTRVQMTWSYPDEKNKNASVRRRIDQSNSHANIFYSVLTIDGMTNSDQGLYTCRVRSGPSFKSVNTSVHIYDEDKTHTCPPCPAPELLGGPSVFLFPPKPKDTLMISRTPEVTCVVVDVSHEDPEVKFNWYVDGVEVHNAKTKPREEQYNSTYRVVSVLTVLHQDWLNGKEYKCKVSNKALPAPIEKTISKAKGQPREPQVYTLPPSREEMTKNQVSLTCLVKGFYPSDIAVEWESNGQPENNYKTTPPVLDSDGSFFLYSKLTVDKSRWQQGNVFSCSVMHEALHNHYTQKSLSLSPGK

SEQ ID NO: 17 - protein, 429 aa, synthetic construct
EFGRPFVEMYSEIPEIIHMTEGRELVIPCRVTSPNITVTLKKFPLDTLIPDGKRIIWDSRKGFIISNATYKEIGLLTCEATVNGHLYKTNYLTHRQTNTIIDVQISTPSPVELSVGETLVLNCTATTPLNTRVQMTWSYPDEKNKNASVRRRIDQSNSHANIFYSVLTIDGMTNSDQGLYTCRVRSGPSFKSVNTSVHIYDEDKTHTCPPCPAPELLGGPSVFLFPPKPKDTLMISRTPEVTCVVVDVSHEDPEVKFNWYVDGVEVHNAKTKPREEQYNSTYRVVSVLTVLHQDWLNGKEYKCKVSNKALPAPIEKTISKAKGQPREPQVYTLPPSREEMTKNQVSLTCLVKGFYPSDIAVEWESNGQPENNYKTTPPVLDSDGSFFLYSKLTVDKSRWQQGNVFSCSVMHEALHNHYTQKSLSLSPGK

SEQ ID NO: 18 - protein, 432 aa, synthetic construct
EFGRPFVEMYSEIPEIIHMTEGRELVIPCRVTSPNITVTLKKFPLDTLIPDGKRIIWDSRKGFIISNATYKEIGLLTCEATVNGHLYKTNYLTHRQTNTIIDVQISTPSPVTLLRGHTLVLNCTATTPSNTRVQMTWSYPDEKNKNASVRRRIDQSNSHANIFYSVLTIDKMQNKDKGLYTCRVRSGPSFKSVNTSVHIYDKALEDKTHTCPPCPAPELLGGPSVFLFPPKPKDTLMISRTPEVTCVVVDVSHEDPEVKFNWYVDGVEVHNAKTKPREEQYNSTYRVVSVLTVLHQDWLNGKEYKCKVSNKALPAPIEKTISKAKGQPREPQVYTLPPSREEMTKNQVSLTCLVKGFYPSDIAVEWESNGQPENNYKTTPPVLDSDGSFFLYSKLTVDKSRWQQGNVFSCSVMHEALHNHYTQKSLSLSPGK

SEQ ID NO: 19 - protein, 432 aa, synthetic construct
EFGRPFVEMYSEIPEIIHMTEGRELVIPCRVTSPNITVTLKKFPLDTLIPDGKRIIWDSRKGFIISNATYKEIGLLTCEATVNGHLYKTNYLTHRQTNTIIDVQISTPSPVTLLRGHTLVLNCTATTPANTRVQMTWSYPDEKNKNASVRRRIDQSNSHANIFYSVLTIDKMQNKDKGLYTCRVRSGPSFKSVNTSVHIYDKALEDKTHTCPPCPAPELLGGPSVFLFPPKPKDTLMISRTPEVTCVVVDVSHEDPEVKFNWYVDGVEVHNAKTKPREEQYNSTYRVVSVLTVLHQDWLNGKEYKCKVSNKALPAPIEKTISKAKGQPREPQVYTLPPSREEMTKNQVSLTCLVKGFYPSDIAVEWESNGQPENNYKTTPPVLDSDGSFFLYSKLTVDKSRWQQGNVFSCSVMHEALHNHYTQKSLSLSPGK

SEQ ID NO: 20 - protein, 429 aa, synthetic construct
EFGRPFVEMYSEIPEIIHMTEGRELVIPCRVTSPNITVTLKKFPLDTLIPDGKRIIWDSRKGFIISNATYKEIGLLTCEATVNGHLYKTNYLTHRQTNTIIDVQISTPSPVELSVGETLVLNCTATTPANTRVQMTWSYPDEKNKNASVRRRIDQSNSHANIFYSVLTIDGMTNSDQGLYTCRVRSGPSFKSVNTSVHIYDEDKTHTCPPCPAPELLGGPSVFLFPPKPKDTLMISRTPEVTCVVVDVSHEDPEVKFNWYVDGVEVHNAKTKPREEQYNSTYRVVSVLTVLHQDWLNGKEYKCKVSNKALPAPIEKTISKAKGQPREPQVYTLPPSREEMTKNQVSLTCLVKGFYPSDIAVEWESNGQPENNYKTTPPVLDSDGSFFLYSKLTVDKSRWQQGNVFSCSVMHEALHNHYTQKSLSLSPGK

SEQ ID NO: 21 - protein, 429 aa, synthetic construct
EFGRPFVEMYSEIPEIIHMTEGRELVIPCRVTSPNITVTLKKFPLDTLIPDGKRIIWDSRKGFIISNATYKEIGLLTCEATVNGHLYKTNYLTHRQTNTIIDVQISTPSPVELSVGETLVLNCTATTPANTRVQMTWSYPDEKNKNASVRRRIDQSNSHANIFYSVLTIDGMQNKDKGLYTCRVRSGPSFKSVNTSVHIYDEDKTHTCPPCPAPELLGGPSVFLFPPKPKDTLMISRTPEVTCVVVDVSHEDPEVKFNWYVDGVEVHNAKTKPREEQYNSTYRVVSVLTVLHQDWLNGKEYKCKVSNKALPAPIEKTISKAKGQPREPQVYTLPPSREEMTKNQVSLTCLVKGFYPSDIAVEWESNGQPENNYKTTPPVLDSDGSFFLYSKLTVDKSRWQQGNVFSCSVMHEALHNHYTQKSLSLSPGK

SEQ ID NO: 22 - protein, 429 aa, synthetic construct
EFGRPFVEMYSEIPEIIHMTEGRELVIPCRVTSPNITVTLKKFPLDTLIPDGKRIIWDSRKGFIISNATYKEIGLLTCEATVNGHLYKTNYLTHRQTNTIIDVQISTPSPVELSVGETLVLNCTATTPANTRVQMTWSYPDEKNKNASVRRRIDQSNSHANIFYSVLTIDGMTNSDKGLYTCRVRSGPSFKSVNTSVHIYDEDKTHTCPPCPAPELLGGPSVFLFPPKPKDTLMISRTPEVTCVVVDVSHEDPEVKFNWYVDGVEVHNAKTKPREEQYNSTYRVVSVLTVLHQDWLNGKEYKCKVSNKALPAPIEKTISKAKGQPREPQVYTLPPSREEMTKNQVSLTCLVKGFYPSDIAVEWESNGQPENNYKTTPPVLDSDGSFFLYSKLTVDKSRWQQGNVFSCSVMHEALHNHYTQKSLSLSPGK

SEQ ID NO: 23 - protein, 429 aa, synthetic construct
EFGRPFVEMYSEIPEIIHMTEGRELVIPCRVTSPNITVTLKKFPLDTLIPDGKRIIWDSRKGFIISNATYKEIGLLTCEATVNGHLYKTNYLTHRQTNTIIDVQISTPSPVTLLRGHTLVLNCTATTPANTRVQMTWSYPDEKNKNASVRRRIDQSNSHANIFYSVLTIDGMTNSDKGLYTCRVRSGPSFKSVNTSVHIYDEDKTHTCPPCPAPELLGGPSVFLFPPKPKDTLMISRTPEVTCVVVDVSHEDPEVKFNWYVDGVEVHNAKTKPREEQYNSTYRVVSVLTVLHQDWLNGKEYKCKVSNKALPAPIEKTISKAKGQPREPQVYTLPPSREEMTKNQVSLTCLVKGFYPSDIAVEWESNGQPENNYKTTPPVLDSDGSFFLYSKLTVDKSRWQQGNVFSCSVMHEALHNHYTQKSLSLSPGK

SEQ ID NO: 24 - protein, 429 aa, synthetic construct
EFGRPFVEMYSEIPEIIHMTEGRELVIPCRVTSPNITVTLKKFPLDTLIPDGKRIIWDSRKGFIISNATYKEIGLLTCEATVNGHLYKTNYLTHRQTNTIIDVQISTPSPVTLLRGHTLVLNCTATTPANTRVQMTWSYPDEKNKNASVRRRIDQSNSHANIFYSVLTIDGMTNSDQGLYTCRVRSGPSFKSVNTSVHIYDEDKTHTCPPCPAPELLGGPSVFLFPPKPKDTLMISRTPEVTCVVVDVSHEDPEVKFNWYVDGVEVHNAKTKPREEQYNSTYRVVSVLTVLHQDWLNGKEYKCKVSNKALPAPIEKTISKAKGQPREPQVYTLPPSREEMTKNQVSLTCLVKGFYPSDIAVEWESNGQPENNYKTTPPVLDSDGSFFLYSKLTVDKSRWQQGNVFSCSVMHEALHNHYTQKSLSLSPGK

SEQ ID NO: 25 - protein, 429 aa, synthetic construct
EFGRPFVEMYSEIPEIIHMTEGRELVIPCRVTSPNITVTLKKFPLDTLIPDGKRIIWDSRKGFIISNATYKEIGLLTCEATVNGHLYKTNYLTHRQTNTIIDVQISTPSPVELSVGETLVLNCTATTPLNTRVQMTWSYPDEKNKNASVRRRIDQSNSHANIFYSVLTIDGMTNSDKGLYTCRVRSGPSFKSVNTSVHIYDEDKTHTCPPCPAPELLGGPSVFLFPPKPKDTLMISRTPEVTCVVVDVSHEDPEVKFNWYVDGVEVHNAKTKPREEQYNSTYRVVSVLTVLHQDWLNGKEYKCKVSNKALPAPIEKTISKAKGQPREPQVYTLPPSREEMTKNQVSLTCLVKGFYPSDIAVEWESNGQPENNYKTTPPVLDSDGSFFLYSKLTVDKSRWQQGNVFSCSVMHEALHNHYTQKSLSLSPGK

SEQ ID NO: 26 - protein, 431 aa, synthetic construct
EFGRPFVEMYSEIPEIIHMTEGRELVIPCRVTSPNITVTLKKFPLDTLIPDGKRIIWDSRKGFIISNATYKEIGLLTCEATVNGHLYKTNYLTHRQTNTIIDVQISTPSPVTLLRGHTLVLNCTATTPLNTRVQMTWSYPDEKNKNASVRRRIDQSNSHANIFYSVLTIDKMQNKDKGLYTCRVRSGPSFKSVNTSVHIYDGSSGDKTHTSPPSPAPELLGGPSVFLFPPKPKDTLMISRTPEVTCVVVDVSHEDPEVKFNWYVDGVEVHNAKTKPREEQYNSTYRVVSVLTVLHQDWLNGKEYKCKVSNKALPAPIEKTISKAKGQPREPQVYTLPPSREEMTKNQVSLTCLVKGFYPSDIAVEWESNGQPENNYKTTPPVLDSDGSFFLYSKLTVDKSRWQQGNVFSCSVMHEALHNHYTQKSLSLSPG

SEQ ID NO: 27 - protein, 436 aa, synthetic construct
EFGRPFVEMYSEIPEIIHMTEGRELVIPCRVTSPNITVTLKKFPLDTLIPDGKRIIWDSRKGFIISNATYKEIGLLTCEATVNGHLYKTNYLTHRQTNTIIDVQISTPSPVTLLRGHTLVLNCTATTPLNTRVQMTWSYPDEKNKNASVRRRIDQSNSHANIFYSVLTIDKMQNKDKGLYTCRVRSGPSFKSVNTSVHIYDGSSGEPKSSDKTYTSPPSPAPELLGGPSVFLFPPKPKDTLMISRTPEVTCVVVDVSHEDPEVKFNWYVDGVEVHNAKTKPREEQYNSTYRVVSVLTVLHQDWLNGKEYKCKVSNKALPAPIEKTISKAKGQPREPQVYTLPPSREEMTKNQVSLTCLVKGFYPSDIAVEWESNGQPENNYKTTPPVLDSDGSFFLYSKLTVDKSRWQQGNVFSCSVMHEALHNHYTQKSLSLSPG

SEQ ID NO: 28 - protein, 440 aa, synthetic construct
EFGRPFVEMYSEIPEIIHMTEGRELVIPCRVTSPNITVTLKKFPLDTLIPDGKRIIWDSRKGFIISNATYKEIGLLTCEATVNGHLYKTNYLTHRQTNTIIDVQISTPSPVTLLRGHTLVLNCTATTPLNTRVQMTWSYPDEKNKNASVRRRIDQSNSHANIFYSVLTIDKMQNKDKGLYTCRVRSGPSFKSVNTSVHIYDGSKVDKKVEPKSSDKTHTCPPCPAPELLGGPSVFLFPPKPKDTLMISRTPEVTCVVVDVSHEDPEVKFNWYVDGVEVHNAKTKPREEQYNSTYRVVSVLTVLHQDWLNGKEYKCKVSNKALPAPIEKTISKAKGQPREPQVYTLPPSREEMTKNQVSLTCLVKGFYPSDIAVEWESNGQPENNYKTTPPVLDSDGSFFLYSKLTVDKSRWQQGNVFSCSVMHEALHNHYTQKSLSLSPG

SEQ ID NO: 29 - protein, 440 aa, synthetic construct
EFGRPFVEMYSEIPEIIHMTEGRELVIPCRVTSPNITVTLKKFPLDTLIPDGKRIIWDSRKGFIISNATYKEIGLLTCEATVNGHLYKTNYLTHRQTNTIIDVQISTPSPVTLLRGHTLVLNCTATTPLNTRVQMTWSYPDEKNKNASVRRRIDQSNSHANIFYSVLTIDKMQNKDKGLYTCRVRSGPSFKSVNTSVHIYDGSKVDKKVEPKSSDKTYTCPPCPAPELLGGPSVFLFPPKPKDTLMISRTPEVTCVVVDVSHEDPEVKFNWYVDGVEVHNAKTKPREEQYNSTYRVVSVLTVLHQDWLNGKEYKCKVSNKALPAPIEKTISKAKGQPREPQVYTLPPSREEMTKNQVSLTCLVKGFYPSDIAVEWESNGQPENNYKTTPPVLDSDGSFFLYSKLTVDKSRWQQGNVFSCSVMHEALHNHYTQKSLSLSPG

SEQ ID NO: 30 - protein, 440 aa, synthetic construct
EFGRPFVEMYSEIPEIIHMTEGRELVIPCRVTSPNITVTLKKFPLDTLIPDGKRIIWDSRKGFIISNATYKEIGLLTCEATVNGHLYKTNYLTHRQTNTIIDVQISTPSPVTLLRGHTLVLNCTATTPLNTRVQMTWSYPDEKNKNASVRRRIDQSNSHANIFYSVLTIDKMQNKDKGLYTCRVRSGPSFKSVNTSVHIYDGSKVDKKVEPKSSDTPPTCPPCPAPELLGGPSVFLFPPKPKDTLMISRTPEVTCVVVDVSHEDPEVKFNWYVDGVEVHNAKTKPREEQYNSTYRVVSVLTVLHQDWLNGKEYKCKVSNKALPAPIEKTISKAKGQPREPQVYTLPPSREEMTKNQVSLTCLVKGFYPSDIAVEWESNGQPENNYKTTPPVLDSDGSFFLYSKLTVDKSRWQQGNVFSCSVMHEALHNHYTQKSLSLSPG

SEQ ID NO: 31 - protein, 447 aa, synthetic construct
EFGRPFVEMYSEIPEIIHMTEGRELVIPCRVTSPNITVTLKKFPLDTLIPDGKRIIWDSRKGFIISNATYKEIGLLTCEATVNGHLYKTNYLTHRQTNTIIDVQISTPSPVTLLRGHTLVLNCTATTPLNTRVQMTWSYPDEKNKNASVRRRIDQSNSHANIFYSVLTIDKMQNKDKGLYTCRVRSGPSFKSVNTSVHIYDGSGGGGSGGGGSGGGGSAESKYGPPCPPCPAPELLGGPSVFLFPPKPKDTLMISRTPEVTCVVVDVSHEDPEVKFNWYVDGVEVHNAKTKPREEQYNSTYRVVSVLTVLHQDWLNGKEYKCKVSNKALPAPIEKTISKAKGQPREPQVYTLPPSREEMTKNQVSLTCLVKGFYPSDIAVEWESNGQPENNYKTTPPVLDSDGSFFLYSKLTVDKSRWQQGNVFSCSVMHEALHNHYTQKSLSLSPG

SEQ ID NO: 32 - protein, 452 aa, synthetic construct
EFGRPFVEMYSEIPEIIHMTEGRELVIPCRVTSPNITVTLKKFPLDTLIPDGKRIIWDSRKGFIISNATYKEIGLLTCEATVNGHLYKTNYLTHRQTNTIIDVQISTPSPVTLLRGHTLVLNCTATTPLNTRVQMTWSYPDEKNKNASVRRRIDQSNSHANIFYSVLTIDKMQNKDKGLYTCRVRSGPSFKSVNTSVHIYDGSNTGSGGEEKKKEKEKEEQEERSSDKTYTCPPCPAPELLGGPSVFLFPPKPKDTLMISRTPEVTCVVVDVSHEDPEVKFNWYVDGVEVHNAKTKPREEQYNSTYRVVSVLTVLHQDWLNGKEYKCKVSNKALPAPIEKTISKAKGQPREPQVYTLPPSREEMTKNQVSLTCLVKGFYPSDIAVEWESNGQPENNYKTTPPVLDSDGSFFLYSKLTVDKSRWQQGNVFSCSVMHEALHNHYTQKSLSLSPG

SEQ ID NO: 33 - protein, 452 aa, synthetic construct
EFGRPFVEMYSEIPEIIHMTEGRELVIPCRVTSPNITVTLKKFPLDTLIPDGKRIIWDSRKGFIISNATYKEIGLLTCEATVNGHLYKTNYLTHRQTNTIIDVQISTPSPVTLLRGHTLVLNCTATTPLNTRVQMTWSYPDEKNKNASVRRRIDQSNSHANIFYSVLTIDKMQNKDKGLYTCRVRSGPSFKSVNTSVHIYDGSNTGSGGEEKKKEKEKEEQEERSSDTPPTCPPCPAPELLGGPSVFLFPPKPKDTLMISRTPEVTCVVVDVSHEDPEVKFNWYVDGVEVHNAKTKPREEQYNSTYRVVSVLTVLHQDWLNGKEYKCKVSNKALPAPIEKTISKAKGQPREPQVYTLPPSREEMTKNQVSLTCLVKGFYPSDIAVEWESNGQPENNYKTTPPVLDSDGSFFLYSKLTVDKSRWQQGNVFSCSVMHEALHNHYTQKSLSLSPG

SEQ ID NO: 34 - protein, 440 aa, synthetic construct
EFGRPFVEMYSEIPEIIHMTEGRELVIPCRVTSPNITVTLKKFPLDTLIPDGKRIIWDSRKGFIISNATYKEIGLLTCEATVNGHLYKTNYLTHRQTNTIIDVQISTPSPVTLLRGHTLVLNCTATTPLNTRVQMTWSYPDEKNKNASVRRRIDQSNSHANIFYSVLTIDKMQNKDKGLYTCRVRSGPSFKSVNTSVHIYDEGSSGGSSGEPKSDATPTCPPCPAPELLGGPSVFLFPPKPKDTLMISRTPEVTCVVVDVSHEDPEVKFNWYVDGVEVHNAKTKPREEQYNSTYRVVSVLTVLHQDWLNGKEYKCKVSNKALPAPIEKTISKAKGQPREPQVYTLPPSREEMTKNQVSLTCLVKGFYPSDIAVEWESNGQPENNYKTTPPVLDSDGSFFLYSKLTVDKSRWQQGNVFSCSVMHEALHNHYTQKSLSLSPG

SEQ ID NO: 35 - protein, 440 aa, synthetic construct
EFGRPFVEMYSEIPEIIHMTEGRELVIPCRVTSPNITVTLKKFPLDTLIPDGKRIIWDSRKGFIISNATYKEIGLLTCEATVNGHLYKTNYLTHRQTNTIIDVQISTPSPVTLLRGHTLVLNCTATTPLNTRVQMTWSYPDEKNKNASVRRRIDQSNSHANIFYSVLTIDKMQNKDKGLYTCRVRSGPSFKSVNTSVHIYDEGSSGGSSGEPKSDSTYTCPPCPAPELLGGPSVFLFPPKPKDTLMISRTPEVTCVVVDVSHEDPEVKFNWYVDGVEVHNAKTKPREEQYNSTYRVVSVLTVLHQDWLNGKEYKCKVSNKALPAPIEKTISKAKGQPREPQVYTLPPSREEMTKNQVSLTCLVKGFYPSDIAVEWESNGQPENNYKTTPPVLDSDGSFFLYSKLTVDKSRWQQGNVFSCSVMHEALHNHYTQKSLSLSPG

SEQ ID NO: 36 - protein, 440 aa, synthetic construct
EFGRPFVEMYSEIPEIIHMTEGRELVIPCRVTSPNITVTLKKFPLDTLIPDGKRIIWDSRKGFIISNATYKEIGLLTCEATVNGHLYKTNYLTHRQTNTIIDVQISTPSPVCLLRGHTLVLNCTATTPLNTRVQMTWSYPDEKNKNASVRRRIDQSNSHANIFYSVLTIDKMQNKDKGLYTCRVRSGPSFKSVNTSVHIYDGCKVDKKVEPKSSDKTYTCPPCPAPELLGGPSVFLFPPKPKDTLMISRTPEVTCVVVDVSHEDPEVKFNWYVDGVEVHNAKTKPREEQYNSTYRVVSVLTVLHQDWLNGKEYKCKVSNKALPAPIEKTISKAKGQPREPQVYTLPPSREEMTKNQVSLTCLVKGFYPSDIAVEWESNGQPENNYKTTPPVLDSDGSFFLYSKLTVDKSRWQQGNVFSCSVMHEALHNHYTQKSLSLSPG

SEQ ID NO: 37 - protein, 440 aa, synthetic construct
EFGRPFVEMYSEIPEIIHMTEGRELVIPCRVTSPNITVTLKKFPLDTLIPDGKRIIWDSRKGFIISNATYKEIGLLTCEATVNGHLYKTNYLTHRQTNTIIDVQISTPSPVTLCRGHTLVLNCTATTPLNTRVQMTWSYPDEKNKNASVRRRIDQSNSHANIFYSVLTIDKMQNKDKGLYTCRVRSGPSFKSVNTSVHICDGSKVDKKVEPKSSDKTYTCPPCPAPELLGGPSVFLFPPKPKDTLMISRTPEVTCVVVDVSHEDPEVKFNWYVDGVEVHNAKTKPREEQYNSTYRVVSVLTVLHQDWLNGKEYKCKVSNKALPAPIEKTISKAKGQPREPQVYTLPPSREEMTKNQVSLTCLVKGFYPSDIAVEWESNGQPENNYKTTPPVLDSDGSFFLYSKLTVDKSRWQQGNVFSCSVMHEALHNHYTQKSLSLSPG

SEQ ID NO: 38 - protein, 440 aa, synthetic construct
EFGRPFVEMYSEIPEIIHMTEGRELVIPCRVTSPNITVTLKKFPLDTLIPDGKRIIWDSRKGFIISNATYKEIGLLTCEATVNGHLYKTNYLTHRQTNTIIDVQISTPSPVTLCRGHTLVLNCTATTPLNTRVQMTWSYPDEKNKNASVRRRIDQSNSHANIFYSVLTIDKMQNKDKGLYTCRVRSGPSFKSVNTSVHIYDCSKVDKKVEPKSSDKTYTCPPCPAPELLGGPSVFLFPPKPKDTLMISRTPEVTCVVVDVSHEDPEVKFNWYVDGVEVHNAKTKPREEQYNSTYRVVSVLTVLHQDWLNGKEYKCKVSNKALPAPIEKTISKAKGQPREPQVYTLPPSREEMTKNQVSLTCLVKGFYPSDIAVEWESNGQPENNYKTTPPVLDSDGSFFLYSKLTVDKSRWQQGNVFSCSVMHEALHNHYTQKSLSLSPG

SEQ ID NO: 39 - protein, 440 aa, synthetic construct
EFGRPFVEMYSEIPEIIHMTEGRELVIPCRVTSPNITVTLKKFPLDTLIPDGKRIIWDSRKGFIISNATYKEIGLLTCEATVNGHLYKTNYLTHRQTNTIIDVQISTPSPVTLLCGHTLVLNCTATTPLNTRVQMTWSYPDEKNKNASVRRRIDQSNSHANIFYSVLTIDKMQNKDKGLYTCRVRSGPSFKSVNTSVHICDGSKVDKKVEPKSSDKTYTCPPCPAPELLGGPSVFLFPPKPKDTLMISRTPEVTCVVVDVSHEDPEVKFNWYVDGVEVHNAKTKPREEQYNSTYRVVSVLTVLHQDWLNGKEYKCKVSNKALPAPIEKTISKAKGQPREPQVYTLPPSREEMTKNQVSLTCLVKGFYPSDIAVEWESNGQPENNYKTTPPVLDSDGSFFLYSKLTVDKSRWQQGNVFSCSVMHEALHNHYTQKSLSLSPG

SEQ ID NO: 40 - protein, 440 aa, synthetic construct
EFGRPFVEMYSEIPEIIHMTEGRELVIPCRVTSPNITVTLKKFPLDTLIPDGKRIIWDSRKGFIISNATYKEIGLLTCEATVNGHLYKTNYLTHRQTNTIIDVQISTPSPVTLLRGHTLVLNCTATTPLNTRVQMTWSYPDEKNKNASVRRRIDQSNSHANIFYSVLTIDKMQCKDKGLYTCRVRSGPSFKSVNTSVHICDGSKVDKKVEPKSSDKTYTCPPCPAPELLGGPSVFLFPPKPKDTLMISRTPEVTCVVVDVSHEDPEVKFNWYVDGVEVHNAKTKPREEQYNSTYRVVSVLTVLHQDWLNGKEYKCKVSNKALPAPIEKTISKAKGQPREPQVYTLPPSREEMTKNQVSLTCLVKGFYPSDIAVEWESNGQPENNYKTTPPVLDSDGSFFLYSKLTVDKSRWQQGNVFSCSVMHEALHNHYTQKSLSLSPG

SEQ ID NO: 41 - protein, 438 aa, synthetic construct
EFGRPFVEMYSEIPEIIHMTEGRELVIPCRVTSPNITVTLKKFPLDTLIPDGKRIIWDSRKGFIISNATYKEIGLLTCEATVNGHLYKTNYLTHRQTNTIIDVQISTPSPVTLLRGHTLVLNCTATTPLNTRVQMTWSYPDEKNKNASVRRRIDQSNSHANIFYSVLTIDKMQNKDKGLYTCRVRSGPSFKSVNTSVHIYDGGGGSAEPKAGDKAPPGPPGPAPELLGGPSVFLFPPKPKDTLMISRTPEVTCVVVDVSHEDPEVKFNWYVDGVEVHNAKTKPREEQYNSTYRVVSVLTVLHQDWLNGKEYKCKVSNKALPAPIEKTISKAKGQPREPQVYTLPPSREEMTKNQVSLTCLVKGFYPSDIAVEWESNGQPENNYKTTPPVLDSDGSFFLYSKLTVDKSRWQQGNVFSCSVMHEALHNHYTQKSLSLSPG

SEQ ID NO: 42 - protein, 438 aa, synthetic construct
EFGRPFVEMYSEIPEIIHMTEGRELVIPCRVTSPNITVTLKKFPLDTLIPDGKRIIWDSRKGFIISNATYKEIGLLTCEATVNGHLYKTNYLTHRQTNTIIDVQISTPSPVTLLRGHTLVLNCTATTPLNTRVQMTWSYPDEKNKNASVRRRIDQSNSHANIFYSVLTIDKMQNKDKGLYTCRVRSGPSFKSVNTSVHIYDGGGGSAEPKSSDKTYTCPPCPAPELLGGPSVFLFPPKPKDTLMISRTPEVTCVVVDVSHEDPEVKFNWYVDGVEVHNAKTKPREEQYNSTYRVVSVLTVLHQDWLNGKEYKCKVSNKALPAPIEKTISKAKGQPREPQVYTLPPSREEMTKNQVSLTCLVKGFYPSDIAVEWESNGQPENNYKTTPPVLDSDGSFFLYSKLTVDKSRWQQGNVFSCSVMHEALHNHYTQKSLSLSPG

SEQ ID NO: 43 - protein, 453 aa, synthetic construct
EFGRPFVEMYSEIPEIIHMTEGRELVIPCRVTSPNITVTLKKFPLDTLIPDGKRIIWDSRKGFIISNATYKEIGLLTCEATVNGHLYKTNYLTHRQTNTIIDVQISTPSPVTLLRGHTLVLNCTATTPLNTRVQMTWSYPDEKNKNASVRRRIDQSNSHANIFYSVLTIDKMQNKDKGLYTCRVRSGPSFKSVNTSVHIYDGGGGSGGGGSGGGGSGGGGSAEPKSSDKTYTCPPCPAPELLGGPSVFLFPPKPKDTLMISRTPEVTCVVVDVSHEDPEVKFNWYVDGVEVHNAKTKPREEQYNSTYRVVSVLTVLHQDWLNGKEYKCKVSNKALPAPIEKTISKAKGQPREPQVYTLPPSREEMTKNQVSLTCLVKGFYPSDIAVEWESNGQPENNYKTTPPVLDSDGSFFLYSKLTVDKSRWQQGNVFSCSVMHEALHNHYTQKSLSLSPG

SEQ ID NO: 44 - protein, 431 aa, synthetic construct
EFGRPFVEMYSEIPEIIHMTEGRELVIPCRVTSPNITVTLKKFPLDTLIPDGKRIIWDSRKGFIISNATYKEIGLLTCEATVNGHLYKTNYLTHRQTNTIIDVQISTPSPVELCVGETLVLNCTATTPANTRVQMTWSYPDEKNKNASVRRRIDQSNSHANIFYSVLTIDGMTNSDKGLYTCRVRSGPSFKSVNTSVHIYDCSSGDATPTSPPSPAPELLGGPSVFLFPPKPKDTLMISRTPEVTCVVVDVSHEDPEVKFNWYVDGVEVHNAKTKPREEQYNSTYRVVSVLTVLHQDWLNGKEYKCKVSNKALPAPIEKTISKAKGQPREPQVYTLPPSRDELTKNQVSLTCLVKGFYPSDIAVEWESNGQPENNYKTTPPVLDSDGSFFLYSKLTVDKSRWQQGNVFSCSVMHEALHNHYTQKSLSLSPG

SEQ ID NO: 45 - protein, 440 aa, synthetic construct
EFGRPFVEMYSEIPEIIHMTEGRELVIPCRVTSPNITVTLKKFPLDTLIPDGKRIIWDSRKGFIISNATYKEIGLLTCEATVNGHLYKTNYLTHRQTNTIIDVQISTPSPVELCVGETLVLNCTATTPANTRVQMTWSYPDEKNKNASVRRRIDQSNSHANIFYSVLTIDGMTNSDKGLYTCRVRSGPSFKSVNTSVHIYDCSKVDKKVEPKSSDTPPTCPPCPAPELLGGPSVFLFPPKPKDTLMISRTPEVTCVVVDVSHEDPEVKFNWYVDGVEVHNAKTKPREEQYNSTYRVVSVLTVLHQDWLNGKEYKCKVSNKALPAPIEKTISKAKGQPREPQVYTLPPSRDELTKNQVSLTCLVKGFYPSDIAVEWESNGQPENNYKTTPPVLDSDGSFFLYSKLTVDKSRWQQGNVFSCSVMHEALHNHYTQKSLSLSPG

SEQ ID NO: 46 - protein, 444 aa, synthetic construct
EFGRPFVEMYSEIPEIIHMTEGRELVIPCRVTSPNITVTLKKFPLDTLIPDGKRIIWDSRKGFIISNATYKEIGLLTCEATVNGHLYKTNYLTHRQTNTIIDVQISTPSPVELCVGETLVLNCTATTPANTRVQMTWSYPDEKNKNASVRRRIDQSNSHANIFYSVLTIDGMTNSDKGLYTCRVRSGPSFKSVNTSVHIYDCSGGGGSAEPKAGDATPPTCPPCPPCPAPELLGGPSVFLFPPKPKDTLMISRTPEVTCVVVDVSHEDPEVKFNWYVDGVEVHNAKTKPREEQYNSTYRVVSVLTVLHQDWLNGKEYKCKVSNKALPAPIEKTISKAKGQPREPQVYTLPPSRDELTKNQVSLTCLVKGFYPSDIAVEWESNGQPENNYKTTPPVLDSDGSFFLYSKLTVDKSRWQQGNVFSCSVMHEALHNHYTQKSLSLSPG

SEQ ID NO: 47 - protein, 447 aa, synthetic construct
EFGRPFVEMYSEIPEIIHMTEGRELVIPCRVTSPNITVTLKKFPLDTLIPDGKRIIWDSRKGFIISNATYKEIGLLTCEATVNGHLYKTNYLTHRQTNTIIDVQISTPSPVELCVGETLVLNCTATTPANTRVQMTWSYPDEKNKNASVRRRIDQSNSHANIFYSVLTIDGMTNSDKGLYTCRVRSGPSFKSVNTSVHIYDCSGGGGSGGGGSGGGGSAESKYGPPCPPCPAPELLGGPSVFLFPPKPKDTLMISRTPEVTCVVVDVSHEDPEVKFNWYVDGVEVHNAKTKPREEQYNSTYRVVSVLTVLHQDWLNGKEYKCKVSNKALPAPIEKTISKAKGQPREPQVYTLPPSRDELTKNQVSLTCLVKGFYPSDIAVEWESNGQPENNYKTTPPVLDSDGSFFLYSKLTVDKSRWQQGNVFSCSVMHEALHNHYTQKSLSLSPG

SEQ ID NO: 48 - protein, 452 aa, synthetic construct
EFGRPFVEMYSEIPEIIHMTEGRELVIPCRVTSPNITVTLKKFPLDTLIPDGKRIIWDSRKGFIISNATYKEIGLLTCEATVNGHLYKTNYLTHRQTNTIIDVQISTPSPVELCVGETLVLNCTATTPANTRVQMTWSYPDEKNKNASVRRRIDQSNSHANIFYSVLTIDGMTNSDKGLYTCRVRSGPSFKSVNTSVHIYDCSNTGSGGEEKKKEKEKEEQEERSSDTPPTCPPCPAPELLGGPSVFLFPPKPKDTLMISRTPEVTCVVVDVSHEDPEVKFNWYVDGVEVHNAKTKPREEQYNSTYRVVSVLTVLHQDWLNGKEYKCKVSNKALPAPIEKTISKAKGQPREPQVYTLPPSRDELTKNQVSLTCLVKGFYPSDIAVEWESNGQPENNYKTTPPVLDSDGSFFLYSKLTVDKSRWQQGNVFSCSVMHEALHNHYTQKSLSLSPG

SEQ ID NO: 49 - protein, 440 aa, synthetic construct
EFGRPFVEMYSEIPEIIHMTEGRELVIPCRVTSPNITVTLKKFPLDTLIPDGKRIIWDSRKGFIISNATYKEIGLLTCEATVNGHLYKTNYLTHRQTNTIIDVQISTPSPVELCVGETLVLNCTATTPANTRVQMTWSYPDEKNKNASVRRRIDQSNSHANIFYSVLTIDGMTNSDKGLYTCRVRSGPSFKSVNTSVHIYDCGSSGGSSGEPKSDATPTCPPCPAPELLGGPSVFLFPPKPKDTLMISRTPEVTCVVVDVSHEDPEVKFNWYVDGVEVHNAKTKPREEQYNSTYRVVSVLTVLHQDWLNGKEYKCKVSNKALPAPIEKTISKAKGQPREPQVYTLPPSRDELTKNQVSLTCLVKGFYPSDIAVEWESNGQPENNYKTTPPVLDSDGSFFLYSKLTVDKSRWQQGNVFSCSVMHEALHNHYTQKSLSLSPG

SEQ ID NO: 50 - protein, 440 aa, synthetic construct
EFGRPFVEMYSEIPEIIHMTEGRELVIPCRVTSPNITVTLKKFPLDTLIPDGKRIIWDSRKGFIISNATYKEIGLLTCEATVNGHLYKTNYLTHRQTNTIIDVQISTPSPVELCVGETLVLNCTATTPANTRVQMTWSYPDEKNKNASVRRRIDQSNSHANIFYSVLTIDGMTNSDKGLYTCRVRSGPSFKSVNTSVHIYDCSKVDKKVEPKSSDKTYTCPPCPAPELLGGPSVFLFPPKPKDTLMISRTPEVTCVVVDVSHEDPEVKFNWYVDGVEVHNAKTKPREEQYNSTYRVVSVLTVLHQDWLNGKEYKCKVSNKALPAPIEKTISKAKGQPREPQVYTLPPSRDELTKNQVSLTCLVKGFYPSDIAVEWESNGQPENNYKTTPPVLDSDGSFFLYSKLTVDKSRWQQGNVFSCSVMHEALHNHYTQKSLSLSPG

SEQ ID NO: 51 - protein, 440 aa, synthetic construct
EFGRPFVEMYSEIPEIIHMTEGRELVIPCRVTSPNITVTLKKFPLDTLIPDGKRIIWDSRKGFIISNATYKEIGLLTCEATVNGHLYKTNYLTHRQTNTIIDVQISTPSPVELCVGETLVLNCTATTPSNTRVQMTWSYPDEKNKNASVRRRIDQSNSHANIFYSVLTIDGMTNSDKGLYTCRVRSGPSFKSVNTSVHIYDCSKVDKKVEPKSSDTPPTCPPCPAPELLGGPSVFLFPPKPKDTLMISRTPEVTCVVVDVSHEDPEVKFNWYVDGVEVHNAKTKPREEQYNSTYRVVSVLTVLHQDWLNGKEYKCKVSNKALPAPIEKTISKAKGQPREPQVYTLPPSRDELTKNQVSLTCLVKGFYPSDIAVEWESNGQPENNYKTTPPVLDSDGSFFLYSKLTVDKSRWQQGNVFSCSVMHEALHNHYTQKSLSLSPG

SEQ ID NO: 52 - protein, 440 aa, synthetic construct
EFGRPFVEMYSEIPEIIHMTEGRELVIPCRVTSPNITVTLKKFPLDTLIPDGKRIIWDSRKGFIISNATYKEIGLLTCEATVNGHLYKTNYLTHRQTNTIIDVQISTPSPVELCVGETLVLNCTATTPDNTRVQMTWSYPDEKNKNASVRRRIDQSNSHANIFYSVLTIDGMTNSDKGLYTCRVRSGPSFKSVNTSVHIYDCSKVDKKVEPKSSDTPPTCPPCPAPELLGGPSVFLFPPKPKDTLMISRTPEVTCVVVDVSHEDPEVKFNWYVDGVEVHNAKTKPREEQYNSTYRVVSVLTVLHQDWLNGKEYKCKVSNKALPAPIEKTISKAKGQPREPQVYTLPPSRDELTKNQVSLTCLVKGFYPSDIAVEWESNGQPENNYKTTPPVLDSDGSFFLYSKLTVDKSRWQQGNVFSCSVMHEALHNHYTQKSLSLSPG

SEQ ID NO: 53 - protein, 447 aa, synthetic construct
EFGRPFVEMYSEIPEIIHMTEGRELVIPCRVTSPNITVTLKKFPLDTLIPDGKRIIWDSRKGFIISNATYKEIGLLTCEATVNGHLYKTNYLTHRQTNTIIDVQISTPSPVELCVGETLVLNCTATTPSNTRVQMTWSYPDEKNKNASVRRRIDQSNSHANIFYSVLTIDGMTNSDKGLYTCRVRSGPSFKSVNTSVHIYDCSGGGGSGGGGSGGGGSAESKYGPPCPPCPAPELLGGPSVFLFPPKPKDTLMISRTPEVTCVVVDVSHEDPEVKFNWYVDGVEVHNAKTKPREEQYNSTYRVVSVLTVLHQDWLNGKEYKCKVSNKALPAPIEKTISKAKGQPREPQVYTLPPSRDELTKNQVSLTCLVKGFYPSDIAVEWESNGQPENNYKTTPPVLDSDGSFFLYSKLTVDKSRWQQGNVFSCSVMHEALHNHYTQKSLSLSPG

SEQ ID NO: 54 - protein, 447 aa, synthetic construct
EFGRPFVEMYSEIPEIIHMTEGRELVIPCRVTSPNITVTLKKFPLDTLIPDGKRIIWDSRKGFIISNATYKEIGLLTCEATVNGHLYKTNYLTHRQTNTIIDVQISTPSPVELCVGETLVLNCTATTPDNTRVQMTWSYPDEKNKNASVRRRIDQSNSHANIFYSVLTIDGMTNSDKGLYTCRVRSGPSFKSVNTSVHIYDCSGGGGSGGGGSGGGGSAESKYGPPCPPCPAPELLGGPSVFLFPPKPKDTLMISRTPEVTCVVVDVSHEDPEVKFNWYVDGVEVHNAKTKPREEQYNSTYRVVSVLTVLHQDWLNGKEYKCKVSNKALPAPIEKTISKAKGQPREPQVYTLPPSRDELTKNQVSLTCLVKGFYPSDIAVEWESNGQPENNYKTTPPVLDSDGSFFLYSKLTVDKSRWQQGNVFSCSVMHEALHNHYTQKSLSLSPG

SEQ ID NO: 55 - protein, 440 aa, synthetic construct
EFGRPFVEMYSEIPEIIHMTEGRELVIPCRVTSPNITVTLKKFPLDTLIPDGKRIIWDSRKGFIISNATYKEIGLLTCEATVNGHLYKTNYLTHRQTNTIIDVQISTPSPVELCVGETLVLNCTATTPSNTRVQMTWSYPDEKNKNASVRRRIDQSNSHANIFYSVLTIDGMTNSDKGLYTCRVRSGPSFKSVNTSVHIYDCGSSGGSSGEPKSDATPTCPPCPAPELLGGPSVFLFPPKPKDTLMISRTPEVTCVVVDVSHEDPEVKFNWYVDGVEVHNAKTKPREEQYNSTYRVVSVLTVLHQDWLNGKEYKCKVSNKALPAPIEKTISKAKGQPREPQVYTLPPSRDELTKNQVSLTCLVKGFYPSDIAVEWESNGQPENNYKTTPPVLDSDGSFFLYSKLTVDKSRWQQGNVFSCSVMHEALHNHYTQKSLSLSPG

SEQ ID NO: 56 - protein, 440 aa, synthetic construct
EFGRPFVEMYSEIPEIIHMTEGRELVIPCRVTSPNITVTLKKFPLDTLIPDGKRIIWDSRKGFIISNATYKEIGLLTCEATVNGHLYKTNYLTHRQTNTIIDVQISTPSPVELCVGETLVLNCTATTPDNTRVQMTWSYPDEKNKNASVRRRIDQSNSHANIFYSVLTIDGMTNSDKGLYTCRVRSGPSFKSVNTSVHIYDCGSSGGSSGEPKSDATPTCPPCPAPELLGGPSVFLFPPKPKDTLMISRTPEVTCVVVDVSHEDPEVKFNWYVDGVEVHNAKTKPREEQYNSTYRVVSVLTVLHQDWLNGKEYKCKVSNKALPAPIEKTISKAKGQPREPQVYTLPPSRDELTKNQVSLTCLVKGFYPSDIAVEWESNGQPENNYKTTPPVLDSDGSFFLYSKLTVDKSRWQQGNVFSCSVMHEALHNHYTQKSLSLSPG

SEQ ID NO: 57 - protein, 431 aa, synthetic construct
EFGRPFVEMYSEIPEIIHMTEGRELVIPCRVTSPNITVTLKKFPLDTLIPDGKRIIWDSRKGFIISNATYKEIGLLTCEATVNGHLYKTNYLTHRQTNTIIDVQISTPSPVELCVGETLVLNCTATTPDNTRVQMTWSYPDEKNKNASVRRRIDQSNSHANIFYSVLTIDGMTNSDKGLYTCRVRSGPSFKSVNTSVHIYDCSSGDATPTSPPSPAPELLGGPSVFLFPPKPKDTLMISRTPEVTCVVVDVSHEDPEVKFNWYVDGVEVHNAKTKPREEQYNSTYRVVSVLTVLHQDWLNGKEYKCKVSNKALPAPIEKTISKAKGQPREPQVYTLPPSRDELTKNQVSLTCLVKGFYPSDIAVEWESNGQPENNYKTTPPVLDSDGSFFLYSKLTVDKSRWQQGNVFSCSVMHEALHNHYTQKSLSLSPG

SEQ ID NO: 58 - protein, 452 aa, synthetic construct
EFGRPFVEMYSEIPEIIHMTEGRELVIPCRVTSPNITVTLKKFPLDTLIPDGKRIIWDSRKGFIISNATYKEIGLLTCEATVNGHLYKTNYLTHRQTNTIIDVQISTPSPVELCVGETLVLNCTATTPDNTRVQMTWSYPDEKNKNASVRRRIDQSNSHANIFYSVLTIDGMTNSDKGLYTCRVRSGPSFKSVNTSVHIYDCSNTGSGGEEKKKEKEKEEQEERSSDTPPTCPPCPAPELLGGPSVFLFPPKPKDTLMISRTPEVTCVVVDVSHEDPEVKFNWYVDGVEVHNAKTKPREEQYNSTYRVVSVLTVLHQDWLNGKEYKCKVSNKALPAPIEKTISKAKGQPREPQVYTLPPSRDELTKNQVSLTCLVKGFYPSDIAVEWESNGQPENNYKTTPPVLDSDGSFFLYSKLTVDKSRWQQGNVFSCSVMHEALHNHYTQKSLSLSPG

SEQ ID NO: 59 - protein, 431 aa, synthetic construct
EFGRPFVEMYSEIPEIIHMTEGRELVIPCRVTSPNITVTLKKFPLDTLIPDGKRIIWDSRKGFIISNATYKEIGLLTCEATVNGHLYKTNYLTHRQTNTIIDVQISTPSPVTLCRGHTLVLNCTATTPANTRVQMTWSYPDEKNKNASVRRRIDQSNSHANIFYSVLTIDGMTNSDQGLYTCRVRSGPSFKSVNTSVHIYDCSSGDATPTSPPSPAPELLGGPSVFLFPPKPKDTLMISRTPEVTCVVVDVSHEDPEVKFNWYVDGVEVHNAKTKPREEQYNSTYRVVSVLTVLHQDWLNGKEYKCKVSNKALPAPIEKTISKAKGQPREPQVYTLPPSRDELTKNQVSLTCLVKGFYPSDIAVEWESNGQPENNYKTTPPVLDSDGSFFLYSKLTVDKSRWQQGNVFSCSVMHEALHNHYTQKSLSLSPG

SEQ ID NO: 60 - protein, 440 aa, synthetic construct
EFGRPFVEMYSEIPEIIHMTEGRELVIPCRVTSPNITVTLKKFPLDTLIPDGKRIIWDSRKGFIISNATYKEIGLLTCEATVNGHLYKTNYLTHRQTNTIIDVQISTPSPVTLCRGHTLVLNCTATTPANTRVQMTWSYPDEKNKNASVRRRIDQSNSHANIFYSVLTIDGMTNSDQGLYTCRVRSGPSFKSVNTSVHIYDCSKVDKKVEPKSSDTPPTCPPCPAPELLGGPSVFLFPPKPKDTLMISRTPEVTCVVVDVSHEDPEVKFNWYVDGVEVHNAKTKPREEQYNSTYRVVSVLTVLHQDWLNGKEYKCKVSNKALPAPIEKTISKAKGQPREPQVYTLPPSRDELTKNQVSLTCLVKGFYPSDIAVEWESNGQPENNYKTTPPVLDSDGSFFLYSKLTVDKSRWQQGNVFSCSVMHEALHNHYTQKSLSLSPG

SEQ ID NO: 61 - protein, 444 aa, synthetic construct
EFGRPFVEMYSEIPEIIHMTEGRELVIPCRVTSPNITVTLKKFPLDTLIPDGKRIIWDSRKGFIISNATYKEIGLLTCEATVNGHLYKTNYLTHRQTNTIIDVQISTPSPVTLCRGHTLVLNCTATTPANTRVQMTWSYPDEKNKNASVRRRIDQSNSHANIFYSVLTIDGMTNSDQGLYTCRVRSGPSFKSVNTSVHIYDCSGGGGSAEPKAGDATPPTCPPCPPCPAPELLGGPSVFLFPPKPKDTLMISRTPEVTCVVVDVSHEDPEVKFNWYVDGVEVHNAKTKPREEQYNSTYRVVSVLTVLHQDWLNGKEYKCKVSNKALPAPIEKTISKAKGQPREPQVYTLPPSRDELTKNQVSLTCLVKGFYPSDIAVEWESNGQPENNYKTTPPVLDSDGSFFLYSKLTVDKSRWQQGNVFSCSVMHEALHNHYTQKSLSLSPG

SEQ ID NO: 62 - protein, 447 aa, synthetic construct
EFGRPFVEMYSEIPEIIHMTEGRELVIPCRVTSPNITVTLKKFPLDTLIPDGKRIIWDSRKGFIISNATYKEIGLLTCEATVNGHLYKTNYLTHRQTNTIIDVQISTPSPVTLCRGHTLVLNCTATTPANTRVQMTWSYPDEKNKNASVRRRIDQSNSHANIFYSVLTIDGMTNSDQGLYTCRVRSGPSFKSVNTSVHIYDCSGGGGSGGGGSGGGGSAESKYGPPCPPCPAPELLGGPSVFLFPPKPKDTLMISRTPEVTCVVVDVSHEDPEVKFNWYVDGVEVHNAKTKPREEQYNSTYRVVSVLTVLHQDWLNGKEYKCKVSNKALPAPIEKTISKAKGQPREPQVYTLPPSRDELTKNQVSLTCLVKGFYPSDIAVEWESNGQPENNYKTTPPVLDSDGSFFLYSKLTVDKSRWQQGNVFSCSVMHEALHNHYTQKSLSLSPG

SEQ ID NO: 63 - protein, 452 aa, synthetic construct
EFGRPFVEMYSEIPEIIHMTEGRELVIPCRVTSPNITVTLKKFPLDTLIPDGKRIIWDSRKGFIISNATYKEIGLLTCEATVNGHLYKTNYLTHRQTNTIIDVQISTPSPVTLCRGHTLVLNCTATTPANTRVQMTWSYPDEKNKNASVRRRIDQSNSHANIFYSVLTIDGMTNSDQGLYTCRVRSGPSFKSVNTSVHIYDCSNTGSGGEEKKKEKEKEEQEERSSDTPPTCPPCPAPELLGGPSVFLFPPKPKDTLMISRTPEVTCVVVDVSHEDPEVKFNWYVDGVEVHNAKTKPREEQYNSTYRVVSVLTVLHQDWLNGKEYKCKVSNKALPAPIEKTISKAKGQPREPQVYTLPPSRDELTKNQVSLTCLVKGFYPSDIAVEWESNGQPENNYKTTPPVLDSDGSFFLYSKLTVDKSRWQQGNVFSCSVMHEALHNHYTQKSLSLSPG

SEQ ID NO: 64 - protein, 440 aa, synthetic construct
EFGRPFVEMYSEIPEIIHMTEGRELVIPCRVTSPNITVTLKKFPLDTLIPDGKRIIWDSRKGFIISNATYKEIGLLTCEATVNGHLYKTNYLTHRQTNTIIDVQISTPSPVTLCRGHTLVLNCTATTPANTRVQMTWSYPDEKNKNASVRRRIDQSNSHANIFYSVLTIDGMTNSDQGLYTCRVRSGPSFKSVNTSVHIYDCGSSGGSSGEPKSDATPTCPPCPAPELLGGPSVFLFPPKPKDTLMISRTPEVTCVVVDVSHEDPEVKFNWYVDGVEVHNAKTKPREEQYNSTYRVVSVLTVLHQDWLNGKEYKCKVSNKALPAPIEKTISKAKGQPREPQVYTLPPSRDELTKNQVSLTCLVKGFYPSDIAVEWESNGQPENNYKTTPPVLDSDGSFFLYSKLTVDKSRWQQGNVFSCSVMHEALHNHYTQKSLSLSPG

SEQ ID NO: 65 - protein, 431 aa, synthetic construct
EFGRPFVEMYSEIPEIIHMTEGRELVIPCRVTSPNITVTLKKFPLDTLIPDGKRIIWDSRKGFIISNATYKEIGLLTCEATVNGHLYKTNYLTHRQTNTIIDVQISTPSPVTLCRGHTLVLNCTATTPDNTRVQMTWSYPDEKNKNASVRRRIDQSNSHANIFYSVLTIDGMTNSDQGLYTCRVRSGPSFKSVNTSVHIYDCSSGDATPTSPPSPAPELLGGPSVFLFPPKPKDTLMISRTPEVTCVVVDVSHEDPEVKFNWYVDGVEVHNAKTKPREEQYNSTYRVVSVLTVLHQDWLNGKEYKCKVSNKALPAPIEKTISKAKGQPREPQVYTLPPSRDELTKNQVSLTCLVKGFYPSDIAVEWESNGQPENNYKTTPPVLDSDGSFFLYSKLTVDKSRWQQGNVFSCSVMHEALHNHYTQKSLSLSPG

SEQ ID NO: 66 - protein, 440 aa, synthetic construct
EFGRPFVEMYSEIPEIIHMTEGRELVIPCRVTSPNITVTLKKFPLDTLIPDGKRIIWDSRKGFIISNATYKEIGLLTCEATVNGHLYKTNYLTHRQTNTIIDVQISTPSPVTLCRGHTLVLNCTATTPDNTRVQMTWSYPDEKNKNASVRRRIDQSNSHANIFYSVLTIDGMTNSDQGLYTCRVRSGPSFKSVNTSVHIYDCSKVDKKVEPKSSDTPPTCPPCPAPELLGGPSVFLFPPKPKDTLMISRTPEVTCVVVDVSHEDPEVKFNWYVDGVEVHNAKTKPREEQYNSTYRVVSVLTVLHQDWLNGKEYKCKVSNKALPAPIEKTISKAKGQPREPQVYTLPPSRDELTKNQVSLTCLVKGFYPSDIAVEWESNGQPENNYKTTPPVLDSDGSFFLYSKLTVDKSRWQQGNVFSCSVMHEALHNHYTQKSLSLSPG

SEQ ID NO: 67 - protein, 444 aa, synthetic construct
EFGRPFVEMYSEIPEIIHMTEGRELVIPCRVTSPNITVTLKKFPLDTLIPDGKRIIWDSRKGFIISNATYKEIGLLTCEATVNGHLYKTNYLTHRQTNTIIDVQISTPSPVTLCRGHTLVLNCTATTPDNTRVQMTWSYPDEKNKNASVRRRIDQSNSHANIFYSVLTIDGMTNSDQGLYTCRVRSGPSFKSVNTSVHIYDCSGGGGSAEPKAGDATPPTCPPCPPCPAPELLGGPSVFLFPPKPKDTLMISRTPEVTCVVVDVSHEDPEVKFNWYVDGVEVHNAKTKPREEQYNSTYRVVSVLTVLHQDWLNGKEYKCKVSNKALPAPIEKTISKAKGQPREPQVYTLPPSRDELTKNQVSLTCLVKGFYPSDIAVEWESNGQPENNYKTTPPVLDSDGSFFLYSKLTVDKSRWQQGNVFSCSVMHEALHNHYTQKSLSLSPG

SEQ ID NO: 68 - protein, 447 aa, synthetic construct
EFGRPFVEMYSEIPEIIHMTEGRELVIPCRVTSPNITVTLKKFPLDTLIPDGKRIIWDSRKGFIISNATYKEIGLLTCEATVNGHLYKTNYLTHRQTNTIIDVQISTPSPVTLCRGHTLVLNCTATTPDNTRVQMTWSYPDEKNKNASVRRRIDQSNSHANIFYSVLTIDGMTNSDQGLYTCRVRSGPSFKSVNTSVHIYDCSGGGGSGGGGSGGGGSAESKYGPPCPPCPAPELLGGPSVFLFPPKPKDTLMISRTPEVTCVVVDVSHEDPEVKFNWYVDGVEVHNAKTKPREEQYNSTYRVVSVLTVLHQDWLNGKEYKCKVSNKALPAPIEKTISKAKGQPREPQVYTLPPSRDELTKNQVSLTCLVKGFYPSDIAVEWESNGQPENNYKTTPPVLDSDGSFFLYSKLTVDKSRWQQGNVFSCSVMHEALHNHYTQKSLSLSPG

SEQ ID NO: 69 - protein, 452 aa, synthetic construct
EFGRPFVEMYSEIPEIIHMTEGRELVIPCRVTSPNITVTLKKFPLDTLIPDGKRIIWDSRKGFIISNATYKEIGLLTCEATVNGHLYKTNYLTHRQTNTIIDVQISTPSPVTLCRGHTLVLNCTATTPDNTRVQMTWSYPDEKNKNASVRRRIDQSNSHANIFYSVLTIDGMTNSDQGLYTCRVRSGPSFKSVNTSVHIYDCSNTGSGGEEKKKEKEKEEQEERSSDTPPTCPPCPAPELLGGPSVFLFPPKPKDTLMISRTPEVTCVVVDVSHEDPEVKFNWYVDGVEVHNAKTKPREEQYNSTYRVVSVLTVLHQDWLNGKEYKCKVSNKALPAPIEKTISKAKGQPREPQVYTLPPSRDELTKNQVSLTCLVKGFYPSDIAVEWESNGQPENNYKTTPPVLDSDGSFFLYSKLTVDKSRWQQGNVFSCSVMHEALHNHYTQKSLSLSPG

SEQ ID NO: 70 - protein, 440 aa, synthetic construct
EFGRPFVEMYSEIPEIIHMTEGRELVIPCRVTSPNITVTLKKFPLDTLIPDGKRIIWDSRKGFIISNATYKEIGLLTCEATVNGHLYKTNYLTHRQTNTIIDVQISTPSPVTLCRGHTLVLNCTATTPDNTRVQMTWSYPDEKNKNASVRRRIDQSNSHANIFYSVLTIDGMTNSDQGLYTCRVRSGPSFKSVNTSVHIYDCGSSGGSSGEPKSDATPTCPPCPAPELLGGPSVFLFPPKPKDTLMISRTPEVTCVVVDVSHEDPEVKFNWYVDGVEVHNAKTKPREEQYNSTYRVVSVLTVLHQDWLNGKEYKCKVSNKALPAPIEKTISKAKGQPREPQVYTLPPSRDELTKNQVSLTCLVKGFYPSDIAVEWESNGQPENNYKTTPPVLDSDGSFFLYSKLTVDKSRWQQGNVFSCSVMHEALHNHYTQKSLSLSPG

SEQ ID NO: 71 - protein, 431 aa, synthetic construct
EFGRPFVEMYSEIPEIIHMTEGRELVIPCRVTSPNITVTLKKFPLDTLIPDGKRIIWDSRKGFIISNATYKEIGLLTCEATVNGHLYKTNYLTHRQTNTIIDVQISTPRPVKLLRGHTLVLNCTATTPLNTRVQMTWSYPDEKNKRASVRRRIDQSNSHANIFYSVLTIDKMQNKDKGLYTCRVRSGPSFKSVNTSVHIYDKALEDKTHTCPPCPAPELLGGPSVFLFPPKPKDTLMISRTPEVTCVVVDVSHEDPEVKFNWYVDGVEVHNAKTKPREEQYNSTYRVVSVLTVLHQDWLNGKEYKCKVSNKALPAPIEKTISKAKGQPREPQVYTLPPSRDELTKNQVSLTCLVKGFYPSDIAVEWESNGQPENNYKTTPPVLDSDGSFFLYSKLTVDKSRWQQGNVFSCSVMHEALHNHYTQKSLSLSPG

SEQ ID NO: 72 - protein, 429 aa, synthetic construct
EFGRPFVEMYSEIPEIIHMTEGRELVIPCRVTSPNITVTLKKFPLDTLIPDGKRIIWDSRKGFIISNATYKEIGLLTCEATVNGHLYKTNYLTHRQTNTIIDVQISTPRPVKLLRGHTLVLNCTATTPLNTRVQMTWSYPDEKNKRASVRRRIDQSNSHANIFYSVLTIDKMQNKDKGLYTCRVRSGPSFKSVNTSVHIYDLEDKTHTCPPCPAPELLGGPSVFLFPPKPKDTLMISRTPEVTCVVVDVSHEDPEVKFNWYVDGVEVHNAKTKPREEQYNSTYRVVSVLTVLHQDWLNGKEYKCKVSNKALPAPIEKTISKAKGQPREPQVYTLPPSRDELTKNQVSLTCLVKGFYPSDIAVEWESNGQPENNYKTTPPVLDSDGSFFLYSKLTVDKSRWQQGNVFSCSVMHEALHNHYTQKSLSLSPG

SEQ ID NO: 73 - protein, 430 aa, synthetic construct
EFGRPFVEMYSEIPEIIHMTEGRELVIPCRVTSPNITVTLKKFPLDTLIPDGKRIIWDSRKGFIISNATYKEIGLLTCEATVNGHLYKTNYLTHRQTNTIIDVQISTPSPVTLLRGHTLVLNCTATTPLNTRVQMTWSYPDEKNKNASVRRRIDQSNSHANIFYSVLTIDKMQNKDKGLYTCRVRSGPSFKSVNTSVHIYDLEDKTHTCPPCPAPELLGGPSVFLFPPKPKDTLMISRTPEVTCVVVDVSHEDPEVKFNWYVDGVEVHNAKTKPREEQYNSTYRVVSVLTVLHQDWLNGKEYKCKVSNKALPAPIEKTISKAKGQPREPQVYTLPPSREEMTKNQVSLTCLVKGFYPSDIAVEWESNGQPENNYKTTPPVLDSDGSFFLYSKLTVDKSRWQQGNVFSCSVMHEALHNHYTQKSLSLSPGK

SEQ ID NO: 74 - protein, 429 aa, synthetic construct
EFGRPFVEMYSEIPEIIHMTEGRELVIPCRVTSPNITVTLKKFPLDTLIPDGKRIIWDSRKGFIISNATYKEIGLLTCEATVNGHLYKTNYLTHRQTNTIIDVQISTPSPVTLLRGHTLVLNCTATTPLNTRVQMTWSYPDEKNKNASVRRRIDQSNSHANIFYSVLTIDKMQNKDKGLYTCRVRSGPSFKSVNTSVHIYDEDKTHTCPPCPAPELLGGPSVFLFPPKPKDTLMISRTPEVTCVVVDVSHEDPEVKFNWYVDGVEVHNAKTKPREEQYNSTYRVVSVLTVLHQDWLNGKEYKCKVSNKALPAPIEKTISKAKGQPREPQVYTLPPSREEMTKNQVSLTCLVKGFYPSDIAVEWESNGQPENNYKTTPPVLDSDGSFFLYSKLTVDKSRWQQGNVFSCSVMHEALHNHYTQKSLSLSPGK

SEQ ID NO: 75 - protein, 432 aa, synthetic construct
EFGRPFVEMYSEIPEIIHMTEGRELVIPCRVTSPNITVTLKKFPLDTLIPDGKRIIWDSRKGFIISNATYKEIGLLTCEATVNGHLYKTNYLTHRQTNTIIDVQISTPSPVTLLRGHTLVLNCTATTPLNTRVQMTWSYPDEKNKNASVRRRIDQSNSHANIFYSVLTIDKMQNKDKGLYTCRVRSGPSFKSVNTSVHIYDKALEDKTHTCPPCPAPELLGGPSVFLFPPKPKDTLMISRTPEVTCVVVDVSHEDPEVKFNWYVDGVEVHNAKTKPREEQYNSTYRVVSVLTVLHQDWLNGKEYKCKVSNKALPAPIEKTISKAKGQPREPQVYTLPPSRDELTKNQVSLTCLVKGFYPSDIAVEWESNGQPENNYKTTPPVLDSDGSFFLYSKLTVDKSRWQQGNVFSCSVMHEALHNHYTQKSLSLSPGK

SEQ ID NO: 76 - protein, 431 aa, synthetic construct
EFGRPFVEMYSEIPEIIHMTEGRELVIPCRVTSPNITVTLKKFPLDTLIPDGKRIIWDSRKGFIISNATYKEIGLLTCEATVNGHLYKTNYLTHRQTNTIIDVQISTPSPVTLLRGHTLVLNCTATTPLNTRVQMTWSYPDEKNKNASVRRRIDQSNSHANIFYSVLTIDKMQNKDKGLYTCRVRSGPSFKSVNTSVHIYDKALEDKTHTCPPCPAPELLGGPSVFLFPPKPKDTLMISRTPEVTCVVVDVSHEDPEVKFNWYVDGVEVHNAKTKPREEQYNSTYRVVSVLTVLHQDWLNGKEYKCKVSNKALPAPIEKTISKAKGQPREPQVYTLPPSREEMTKNQVSLTCLVKGFYPSDIAVEWESNGQPENNYKTTPPVLDSDGSFFLYSKLTVDKSRWQQGNVFSCSVMHEALHNHYTQKSLSLSPG

SEQ ID NO: 77 - protein, 429 aa, synthetic construct
EFGRPFVEMYSEIPEIIHMTEGRELVIPCRVTSPNITVTLKKFPLDTLIPDGKRIIWDSRKGFIISNATYKEIGLLTCEATVNGHLYKTNYLTHRQTNTIIDVQISTPRPVKLSVGHTLVLNCTATTPLNTRVQMTWSYPDEKNKRASVRRRIDQSNSHANIFYSVLTIDKMQNKDKGLYTCRVRSGPSFKSVNTSVHIYDLEDKTHTCPPCPAPELLGGPSVFLFPPKPKDTLMISRTPEVTCVVVDVSHEDPEVKFNWYVDGVEVHNAKTKPREEQYNSTYRVVSVLTVLHQDWLNGKEYKCKVSNKALPAPIEKTISKAKGQPREPQVYTLPPSRDELTKNQVSLTCLVKGFYPSDIAVEWESNGQPENNYKTTPPVLDSDGSFFLYSKLTVDKSRWQQGNVFSCSVMHEALHNHYTQKSLSLSPG

SEQ ID NO: 78 - protein, 429 aa, synthetic construct
EFGRPFVEMYSEIPEIIHMTEGRELVIPCRVTSPNITVTLKKFPLDTLIPDGKRIIWDSRKGFIISNATYKEIGLLTCEATVNGHLYKTNYLTHRQTNTIIDVQISTPRPVELSVGETLVLNCTATTPLNTRVQMTWSYPDEKNKRASVRRRIDQSNSHANIFYSVLTIDKMQNKDKGLYTCRVRSGPSFKSVNTSVHIYDLEDKTHTCPPCPAPELLGGPSVFLFPPKPKDTLMISRTPEVTCVVVDVSHEDPEVKFNWYVDGVEVHNAKTKPREEQYNSTYRVVSVLTVLHQDWLNGKEYKCKVSNKALPAPIEKTISKAKGQPREPQVYTLPPSRDELTKNQVSLTCLVKGFYPSDIAVEWESNGQPENNYKTTPPVLDSDGSFFLYSKLTVDKSRWQQGNVFSCSVMHEALHNHYTQKSLSLSPG

SEQ ID NO: 79 - protein, 429 aa, synthetic construct
EFGRPFVEMYSEIPEIIHMTEGRELVIPCRVTSPNITVTLKKFPLDTLIPDGKRIIWDSRKGFIISNATYKEIGLLTCEATVNGHLYKTNYLTHRQTNTIIDVQISTPRPVKLLRGHTLVLNCTATTPANTRVQMTWSYPDEKNKRASVRRRIDQSNSHANIFYSVLTIDKMQNKDKGLYTCRVRSGPSFKSVNTSVHIYDLEDKTHTCPPCPAPELLGGPSVFLFPPKPKDTLMISRTPEVTCVVVDVSHEDPEVKFNWYVDGVEVHNAKTKPREEQYNSTYRVVSVLTVLHQDWLNGKEYKCKVSNKALPAPIEKTISKAKGQPREPQVYTLPPSRDELTKNQVSLTCLVKGFYPSDIAVEWESNGQPENNYKTTPPVLDSDGSFFLYSKLTVDKSRWQQGNVFSCSVMHEALHNHYTQKSLSLSPG

SEQ ID NO: 80 - protein, 429 aa, synthetic construct
EFGRPFVEMYSEIPEIIHMTEGRELVIPCRVTSPNITVTLKKFPLDTLIPDGKRIIWDSRKGFIISNATYKEIGLLTCEATVNGHLYKTNYLTHRQTNTIIDVQISTPRPVKLLRGHTLVLNCTATTPLNTRVQMTWSYPDEKNKRASVRRRIDQSNSHANIFYSVLTIDGMTNSDQGLYTCRVRSGPSFKSVNTSVHIYDLEDKTHTCPPCPAPELLGGPSVFLFPPKPKDTLMISRTPEVTCVVVDVSHEDPEVKFNWYVDGVEVHNAKTKPREEQYNSTYRVVSVLTVLHQDWLNGKEYKCKVSNKALPAPIEKTISKAKGQPREPQVYTLPPSRDELTKNQVSLTCLVKGFYPSDIAVEWESNGQPENNYKTTPPVLDSDGSFFLYSKLTVDKSRWQQGNVFSCSVMHEALHNHYTQKSLSLSPG

SEQ ID NO: 81 - protein, 429 aa, synthetic construct
EFGRPFVEMYSEIPEIIHMTEGRELVIPCRVTSPNITVTLKKFPLDTLIPDGKRIIWDSRKGFIISNATYKEIGLLTCEATVNGHLYKTNYLTHRQTNTIIDVQISTPRPVKLSVGHTLVLNCTATTPANTRVQMTWSYPDEKNKRASVRRRIDQSNSHANIFYSVLTIDKMQNKDKGLYTCRVRSGPSFKSVNTSVHIYDLEDKTHTCPPCPAPELLGGPSVFLFPPKPKDTLMISRTPEVTCVVVDVSHEDPEVKFNWYVDGVEVHNAKTKPREEQYNSTYRVVSVLTVLHQDWLNGKEYKCKVSNKALPAPIEKTISKAKGQPREPQVYTLPPSRDELTKNQVSLTCLVKGFYPSDIAVEWESNGQPENNYKTTPPVLDSDGSFFLYSKLTVDKSRWQQGNVFSCSVMHEALHNHYTQKSLSLSPG

SEQ ID NO: 82 - protein, 429 aa, synthetic construct
EFGRPFVEMYSEIPEIIHMTEGRELVIPCRVTSPNITVTLKKFPLDTLIPDGKRIIWDSRKGFIISNATYKEIGLLTCEATVNGHLYKTNYLTHRQTNTIIDVQISTPRPVKLLRGHTLVLNCTATTPANTRVQMTWSYPDEKNKRASVRRRIDQSNSHANIFYSVLTIDGMTNSDKGLYTCRVRSGPSFKSVNTSVHIYDLEDKTHTCPPCPAPELLGGPSVFLFPPKPKDTLMISRTPEVTCVVVDVSHEDPEVKFNWYVDGVEVHNAKTKPREEQYNSTYRVVSVLTVLHQDWLNGKEYKCKVSNKALPAPIEKTISKAKGQPREPQVYTLPPSRDELTKNQVSLTCLVKGFYPSDIAVEWESNGQPENNYKTTPPVLDSDGSFFLYSKLTVDKSRWQQGNVFSCSVMHEALHNHYTQKSLSLSPG

SEQ ID NO: 83 - protein, 429 aa, synthetic construct
EFGRPFVEMYSEIPEIIHMTEGRELVIPCRVTSPNITVTLKKFPLDTLIPDGKRIIWDSRKGFIISNATYKEIGLLTCEATVNGHLYKTNYLTHRQTNTIIDVQISTPRPVKLLRGHTLVLNCTATTPANTRVQMTWSYPDEKNKRASVRRRIDQSNSHANIFYSVLTIDGMTNSDQGLYTCRVRSGPSFKSVNTSVHIYDLEDKTHTCPPCPAPELLGGPSVFLFPPKPKDTLMISRTPEVTCVVVDVSHEDPEVKFNWYVDGVEVHNAKTKPREEQYNSTYRVVSVLTVLHQDWLNGKEYKCKVSNKALPAPIEKTISKAKGQPREPQVYTLPPSRDELTKNQVSLTCLVKGFYPSDIAVEWESNGQPENNYKTTPPVLDSDGSFFLYSKLTVDKSRWQQGNVFSCSVMHEALHNHYTQKSLSLSPG

SEQ ID NO: 84 - protein, 429 aa, synthetic construct
EFGRPFVEMYSEIPEIIHMTEGRELVIPCRVTSPNITVTLKKFPLDTLIPDGKRIIWDSRKGFIISNATYKEIGLLTCEATVNGHLYKTNYLTHRQTNTIIDVQISTPRPVELSVGETLVLNCTATTPLNTRVQMTWSYPDEKNKRASVRRRIDQSNSHANIFYSVLTIDGMTNSDQGLYTCRVRSGPSFKSVNTSVHIYDLEDKTHTCPPCPAPELLGGPSVFLFPPKPKDTLMISRTPEVTCVVVDVSHEDPEVKFNWYVDGVEVHNAKTKPREEQYNSTYRVVSVLTVLHQDWLNGKEYKCKVSNKALPAPIEKTISKAKGQPREPQVYTLPPSRDELTKNQVSLTCLVKGFYPSDIAVEWESNGQPENNYKTTPPVLDSDGSFFLYSKLTVDKSRWQQGNVFSCSVMHEALHNHYTQKSLSLSPG

SEQ ID NO: 85 - protein, 429 aa, synthetic construct
EFGRPFVEMYSEIPEIIHMTEGRELVIPCRVTSPNITVTLKKFPLDTLIPDGKRIIWDSRKGFIISNATYKEIGLLTCEATVNGHLYKTNYLTHRQTNTIIDVQISTPRPVELSVGETLVLNCTATTPANTRVQMTWSYPDEKNKRASVRRRIDQSNSHANIFYSVLTIDGMTNSDQGLYTCRVRSGPSFKSVNTSVHIYDLEDKTHTCPPCPAPELLGGPSVFLFPPKPKDTLMISRTPEVTCVVVDVSHEDPEVKFNWYVDGVEVHNAKTKPREEQYNSTYRVVSVLTVLHQDWLNGKEYKCKVSNKALPAPIEKTISKAKGQPREPQVYTLPPSRDELTKNQVSLTCLVKGFYPSDIAVEWESNGQPENNYKTTPPVLDSDGSFFLYSKLTVDKSRWQQGNVFSCSVMHEALHNHYTQKSLSLSPG

SEQ ID NO: 86 - protein, 429 aa, synthetic construct
EFGRPFVEMYSEIPEIIHMTEGRELVIPCRVTSPNITVTLKKFPLDTLIPDGKRIIWDSRKGFIISNATYKEIGLLTCEATVNGHLYKTNYLTHRQTNTIIDVQISTPRPVELSVGETLVLNCTATTPANTRVQMTWSYPDEKNKRASVRRRIDQSNSHANIFYSVLTIDGMQNKDKGLYTCRVRSGPSFKSVNTSVHIYDLEDKTHTCPPCPAPELLGGPSVFLFPPKPKDTLMISRTPEVTCVVVDVSHEDPEVKFNWYVDGVEVHNAKTKPREEQYNSTYRVVSVLTVLHQDWLNGKEYKCKVSNKALPAPIEKTISKAKGQPREPQVYTLPPSRDELTKNQVSLTCLVKGFYPSDIAVEWESNGQPENNYKTTPPVLDSDGSFFLYSKLTVDKSRWQQGNVFSCSVMHEALHNHYTQKSLSLSPG

SEQ ID NO: 87 - protein, 429 aa, synthetic construct
EFGRPFVEMYSEIPEIIHMTEGRELVIPCRVTSPNITVTLKKFPLDTLIPDGKRIIWDSRKGFIISNATYKEIGLLTCEATVNGHLYKTNYLTHRQTNTIIDVQISTPRPVELSVGETLVLNCTATTPANTRVQMTWSYPDEKNKRASVRRRIDQSNSHANIFYSVLTIDGMTNSDKGLYTCRVRSGPSFKSVNTSVHIYDLEDKTHTCPPCPAPELLGGPSVFLFPPKPKDTLMISRTPEVTCVVVDVSHEDPEVKFNWYVDGVEVHNAKTKPREEQYNSTYRVVSVLTVLHQDWLNGKEYKCKVSNKALPAPIEKTISKAKGQPREPQVYTLPPSRDELTKNQVSLTCLVKGFYPSDIAVEWESNGQPENNYKTTPPVLDSDGSFFLYSKLTVDKSRWQQGNVFSCSVMHEALHNHYTQKSLSLSPG

SEQ ID NO: 88 - protein, 431 aa, synthetic construct
EFGRPFVEMYSEIPEIIHMTEGRELVIPCRVTSPNITVTLKKFPLDTLIPDGKRIIWDSRKGFIISNATYKEIGLLTCEATVNGHLYKTNYLTHRQTNTIIDVQISTPRPVKLLRGHTLVLNCTATTPLNTRVQMTWSYPDEKNKRASVRRRIDQSNSHANIFYSVLTIDKMQNKDKGLYTCRVRSGPSFKSVNTSVHIYDGSSGDKTHTSPPSPAPELLGGPSVFLFPPKPKDTLMISRTPEVTCVVVDVSHEDPEVKFNWYVDGVEVHNAKTKPREEQYNSTYRVVSVLTVLHQDWLNGKEYKCKVSNKALPAPIEKTISKAKGQPREPQVYTLPPSRDELTKNQVSLTCLVKGFYPSDIAVEWESNGQPENNYKTTPPVLDSDGSFFLYSKLTVDKSRWQQGNVFSCSVMHEALHNHYTQKSLSLSPG

SEQ ID NO: 89 - protein, 440 aa, synthetic construct
EFGRPFVEMYSEIPEIIHMTEGRELVIPCRVTSPNITVTLKKFPLDTLIPDGKRIIWDSRKGFIISNATYKEIGLLTCEATVNGHLYKTNYLTHRQTNTIIDVQISTPRPVKLLRGHTLVLNCTATTPLNTRVQMTWSYPDEKNKRASVRRRIDQSNSHANIFYSVLTIDKMQNKDKGLYTCRVRSGPSFKSVNTSVHIYDGSKVDKKVEPKSSDKTHTCPPCPAPELLGGPSVFLFPPKPKDTLMISRTPEVTCVVVDVSHEDPEVKFNWYVDGVEVHNAKTKPREEQYNSTYRVVSVLTVLHQDWLNGKEYKCKVSNKALPAPIEKTISKAKGQPREPQVYTLPPSRDELTKNQVSLTCLVKGFYPSDIAVEWESNGQPENNYKTTPPVLDSDGSFFLYSKLTVDKSRWQQGNVFSCSVMHEALHNHYTQKSLSLSPG

SEQ ID NO: 90 - protein, 440 aa, synthetic construct
EFGRPFVEMYSEIPEIIHMTEGRELVIPCRVTSPNITVTLKKFPLDTLIPDGKRIIWDSRKGFIISNATYKEIGLLTCEATVNGHLYKTNYLTHRQTNTIIDVQISTPRPVKLLRGHTLVLNCTATTPLNTRVQMTWSYPDEKNKRASVRRRIDQSNSHANIFYSVLTIDKMQNKDKGLYTCRVRSGPSFKSVNTSVHIYDEGSSGGSSGEPKSDATPTCPPCPAPELLGGPSVFLFPPKPKDTLMISRTPEVTCVVVDVSHEDPEVKFNWYVDGVEVHNAKTKPREEQYNSTYRVVSVLTVLHQDWLNGKEYKCKVSNKALPAPIEKTISKAKGQPREPQVYTLPPSRDELTKNQVSLTCLVKGFYPSDIAVEWESNGQPENNYKTTPPVLDSDGSFFLYSKLTVDKSRWQQGNVFSCSVMHEALHNHYTQKSLSLSPG

SEQ ID NO: 91 - protein, 440 aa, synthetic construct
EFGRPFVEMYSEIPEIIHMTEGRELVIPCRVTSPNITVTLKKFPLDTLIPDGKRIIWDSRKGFIISNATYKEIGLLTCEATVNGHLYKTNYLTHRQTNTIIDVQISTPRPVKLCRGHTLVLNCTATTPLNTRVQMTWSYPDEKNKRASVRRRIDQSNSHANIFYSVLTIDKMQNKDKGLYTCRVRSGPSFKSVNTSVHIYDCSKVDKKVEPKSSDKTYTCPPCPAPELLGGPSVFLFPPKPKDTLMISRTPEVTCVVVDVSHEDPEVKFNWYVDGVEVHNAKTKPREEQYNSTYRVVSVLTVLHQDWLNGKEYKCKVSNKALPAPIEKTISKAKGQPREPQVYTLPPSRDELTKNQVSLTCLVKGFYPSDIAVEWESNGQPENNYKTTPPVLDSDGSFFLYSKLTVDKSRWQQGNVFSCSVMHEALHNHYTQKSLSLSPG

SEQ ID NO: 92 - protein, 452 aa, synthetic construct
EFGRPFVEMYSEIPEIIHMTEGRELVIPCRVTSPNITVTLKKFPLDTLIPDGKRIIWDSRKGFIISNATYKEIGLLTCEATVNGHLYKTNYLTHRQTNTIIDVQISTPRPVELCVGETLVLNCTATTPANTRVQMTWSYPDEKNKRASVRRRIDQSNSHANIFYSVLTIDGMTNSDKGLYTCRVRSGPSFKSVNTSVHIYDCSNTGSGGEEKKKEKEKEEQEERSSDTPPTCPPCPAPELLGGPSVFLFPPKPKDTLMISRTPEVTCVVVDVSHEDPEVKFNWYVDGVEVHNAKTKPREEQYNSTYRVVSVLTVLHQDWLNGKEYKCKVSNKALPAPIEKTISKAKGQPREPQVYTLPPSRDELTKNQVSLTCLVKGFYPSDIAVEWESNGQPENNYKTTPPVLDSDGSFFLYSKLTVDKSRWQQGNVFSCSVMHEALHNHYTQKSLSLSPG

SEQ ID NO: 93 - protein, 440 aa, synthetic construct
EFGRPFVEMYSEIPEIIHMTEGRELVIPCRVTSPNITVTLKKFPLDTLIPDGKRIIWDSRKGFIISNATYKEIGLLTCEATVNGHLYKTNYLTHRQTNTIIDVQISTPRPVELCVGETLVLNCTATTPDNTRVQMTWSYPDEKNKRASVRRRIDQSNSHANIFYSVLTIDGMTNSDKGLYTCRVRSGPSFKSVNTSVHIYDCGSSGGSSGEPKSDATPTCPPCPAPELLGGPSVFLFPPKPKDTLMISRTPEVTCVVVDVSHEDPEVKFNWYVDGVEVHNAKTKPREEQYNSTYRVVSVLTVLHQDWLNGKEYKCKVSNKALPAPIEKTISKAKGQPREPQVYTLPPSRDELTKNQVSLTCLVKGFYPSDIAVEWESNGQPENNYKTTPPVLDSDGSFFLYSKLTVDKSRWQQGNVFSCSVMHEALHNHYTQKSLSLSPG

SEQ ID NO: 94 - protein, 419 aa, synthetic construct
EFGRPFVEMYSEIPEIIHMTEGRELVIPCRVTSPNITVTLKKFPLDTLIPDGKRIIWDSRKGFIISNATYKEIGLLTCEATVNGHLYKTNYLTHRQTNTIIDVQISTPRPVKLLRGHTLVLNCTATTPLNTRVQMTWSYPDEKNKRASVRRRIDQSNSHANIFYSVLTIDKMQNKDKGLYTCRVRSGPSFKSVNTSVHIYDKAAPELLGGPSVFLFPPKPKDTLMISRTPEVTCVVVDVSHEDPEVKFNWYVDGVEVHNAKTKPREEQYNSTYRVVSVLTVLHQDWLNGKEYKCKVSNKALPAPIEKTISKAKGQPREPQVYTLPPSRDELTKNQVSLTCLVKGFYPSDIAVEWESNGQPENNYKTTPPVLDSDGSFFLYSKLTVDKSRWQQGNVFSCSVMHEALHNHYTQKSLSLSPG

SEQ ID NO: 95 - protein, 469 aa, synthetic construct
EFGRPFVEMYSEIPEIIHMTEGRELVIPCRVTSPNITVTLKKFPLDTLIPDGKRIIWDSRKGFIISNATYKEIGLLTCEATVNGHLYKTNYLTHRQTNTIIDVQISTPRPVKLLRGHTLVLNCTATTPLNTRVQMTWSYPDEKNKRASVRRRIDQSNSHANIFYSVLTIDKMQNKDKGLYTCRVRSGPSFKSVNTSVHIYDKAGSSGGSSGGSSGGSSGGSSGGSSGGSSGGSSGGSSGGSSGDKTHTCPPCPAPELLGGPSVFLFPPKPKDTLMISRTPEVTCVVVDVSHEDPEVKFNWYVDGVEVHNAKTKPREEQYNSTYRVVSVLTVLHQDWLNGKEYKCKVSNKALPAPIEKTISKAKGQPREPQVYTLPPSRDELTKNQVSLTCLVKGFYPSDIAVEWESNGQPENNYKTTPPVLDSDGSFFLYSKLTVDKSRWQQGNVFSCSVMHEALHNHYTQKSLSLSPG

SEQ ID NO: 96 - protein, 469 aa, synthetic construct
EFGRPFVEMYSEIPEIIHMTEGRELVIPCRVTSPNITVTLKKFPLDTLIPDGKRIIWDSRKGFIISNATYKEIGLLTCEATVNGHLYKTNYLTHRQTNTIIDVQISTPRPVKLLRGHTLVLNCTATTPLNTRVQMTWSYPDEKNKRASVRRRIDQSNSHANIFYSVLTIDKMQNKDKGLYTCRVRSGPSFKSVNTSVHIYDKAGGGGSGGGGSGGGGSGGGGSGGGGSGGGGSGGGGSGGGGSDKTHTCPPCPAPELLGGPSVFLFPPKPKDTLMISRTPEVTCVVVDVSHEDPEVKFNWYVDGVEVHNAKTKPREEQYNSTYRVVSVLTVLHQDWLNGKEYKCKVSNKALPAPIEKTISKAKGQPREPQVYTLPPSRDELTKNQVSLTCLVKGFYPSDIAVEWESNGQPENNYKTTPPVLDSDGSFFLYSKLTVDKSRWQQGNVFSCSVMHEALHNHYTQKSLSLSPG

SEQ ID NO: 97 - protein, 459 aa, synthetic construct
EFGRPFVEMYSEIPEIIHMTEGRELVIPCRVTSPNITVTLKKFPLDTLIPDGKRIIWDSRKGFIISNATYKEIGLLTCEATVNGHLYKTNYLTHRQTNTIIDVQISTPRPVKLLRGHTLVLNCTATTPLNTRVQMTWSYPDEKNKRASVRRRIDQSNSHANIFYSVLTIDKMQNKDKGLYTCRVRSGPSFKSVNTSVHIYDKAGGGGSGGGGSGGGGSGGGGSGGGGSGGGGSDKTHTCPPCPAPELLGGPSVFLFPPKPKDTLMISRTPEVTCVVVDVSHEDPEVKFNWYVDGVEVHNAKTKPREEQYNSTYRVVSVLTVLHQDWLNGKEYKCKVSNKALPAPIEKTISKAKGQPREPQVYTLPPSRDELTKNQVSLTCLVKGFYPSDIAVEWESNGQPENNYKTTPPVLDSDGSFFLYSKLTVDKSRWQQGNVFSCSVMHEALHNHYTQKSLSLSPG

SEQ ID NO: 98 - protein, 429 aa, synthetic construct
EFGRPFVEMYSEIPEIIHMTEGRELVIPCRVTSPNITVTLKKFPLDTLIPDGKRIIWDSRKGFIISNATYKEIGLLTCEATVNGHLYKTNYLTHRQTNTIIDVQISTPRPVKLLRGHTLVLNCTATTPDNTRVQMTWSYPDEKNKRASVRRRIDQSNSHANIFYSVLTIDKMQNKDKGLYTCRVRSGPSFKSVNTSVHIYDLEDKTHTCPPCPAPELLGGPSVFLFPPKPKDTLMISRTPEVTCVVVDVSHEDPEVKFNWYVDGVEVHNAKTKPREEQYNSTYRVVSVLTVLHQDWLNGKEYKCKVSNKALPAPIEKTISKAKGQPREPQVYTLPPSRDELTKNQVSLTCLVKGFYPSDIAVEWESNGQPENNYKTTPPVLDSDGSFFLYSKLTVDKSRWQQGNVFSCSVMHEALHNHYTQKSLSLSPG

SEQ ID NO: 99 - protein, 217 aa, Homo sapiens
APELLGGPSVFLFPPKPKDTLMISRTPEVTCVVVDVSHEDPEVKFNWYVDGVEVHNAKTKPREEQYNSTYRVVSVLTVLHQDWLNGKEYKCKVSNKALPAPIEKTISKAKGQPREPQVYTLPPSRDELTKNQVSLTCLVKGFYPSDIAVEWESNGQPENNYKTTPPVLDSDGSFFLYSKLTVDKSRWQQGNVFSCSVMHEALHNHYTQKSLSLSPGK

SEQ ID NO: 100 - protein, 201 aa, Homo sapiens
  DOMAIN 84..201: note = domain D3
  DOMAIN 1..83: note = domain D2
  SITE 1: note = G132 of VEGFR1
  SITE 84: note = L215 of VEGFR1
GRPFVEMYSEIPEIIHMTEGRELVIPCRVTSPNITVTLKKFPLDTLIPDGKRIIWDSRKGFIISNATYKEIGLLTCEATVNGHLYKTNYLTHRQTNTIIDVQISTPRPVKLLRGHTLVLNCTATTPLNTRVQMTWSYPDEKNKRASVRRRIDQSNSHANIFYSVLTIDKMQNKDKGLYTCRVRSGPSFKSVNTSVHIYDKA

SEQ ID NO: 101 - protein, 433 aa, synthetic construct
SDTGRPFVEMYSEIPEIIHMTEGRELVIPCRVTSPNITVTLKKFPLDTLIPDGKRIIWDSRKGFIISNATYKEIGLLTCEATVNGHLYKTNYLTHRQTNTIIDVVLSPSHGIELSVGEKLVLNCTARTELNVGIDFNWEYPSSKHQHKKLVNRDLKTQSGSEMKKFLSTLTIDGVTRSDQGLYTCAASSGLMTKKNSTFVRVHEKLEDKTHTCPPCPAPELLGGPSVFLFPPKPKDTLMISRTPEVTCVVVDVSHEDPEVKFNWYVDGVEVHNAKTKPREEQYNSTYRVVSVLTVLHQDWLNGKEYKCKVSNKALPAPIEKTISKAKGQPREPQVYTLPPSRDELTKNQVSLTCLVKGFYPSDIAVEWESNGQPENNYKTTPPVLDSDGSFFLYSKLTVDKSRWQQGNVFSCSVMHEALHNHYTQKSLSLSPG